European Patent Specification EP 3 227 438 B1, published March 27, 2024. Title: Laccase Variants and Polynucleotides Encoding Same. Applicant: Novozymes A/S Held, Daniel Luttringer, Sheryl Doty, Tammy. The sequence listing filed with the application follows.

SEQUENCE LISTING (95 sequences)

SEQ ID NO: 1 - DNA, 1563 bp, Polyporus pinsitus
atgtcgaggtttcactctcttctcgctttcgtcgttgcttcccttacggctgtggcccacgctggtatcggtcccgtcgccgacctaaccatcaccaacgcagcggtcagccccgacgggttttctcgccaggccgtcgtcgtgaacggcggcacccctggccctctcatcaccggtaacatgggggatcgcttccagctcaatgtcatcgacaaccttaccaaccacacgatgctgaagagcacgagtattcactggcacggtttcttccagaagggtaccaactgggccgacggtcccgccttcatcaaccagtgcccgatctcatctggtcactcgttcctgtacgacttccaggttcctgaccaggctggtaccttctggtatcacagtcacttgtctacgcagtactgtgatggtttgaggggtccgttcgttgtttacgacccgaatgacccggccgccgacctgtacgacgtcgacaacgacgacactgtcattacccttgtggattggtaccacgtcgccgcgaagctgggccccgcattccctctcggcgccgacgccaccctcatcaacggtaagggacgctcccccagcacgaccaccgcggacctctcagttatcagcgtcaccccgggtaaacgctaccgtttccgcctggtgtccctgtcgtgcgaccccaactacacgttcagcatcgatggtcacaacatgacgatcatcgagaccgactcaatcaacacggcgcccctcgtcgtcgactccattcagatcttcgccgcccagcgttactccttcgtgctcgaggccaaccaggccgtcgacaactactggattcgcgccaacccgaacttcggtaacgtcgggttcaccggcggcattaactcggctatcctccgctacgatggtgccgctgccgtggagcccaccaccacgcaaaccacgtcgactgcgccgctcaacgaggtcaacctgcacccgctggttaccaccgctgtgcctggctcgcccgtcgctggtggtgtcgacctggccatcaacatggcgttcaacttcaacggcaccaacttcttcatcaacggcgcgtctttcacgcccccgaccgtgcctgtcctgctccagatcatcagcggcgcgcagaacgcgcaggacctcctgccctccggtagcgtctactcgcttccctcgaacgccgacatcgagatctccttccccgccaccgccgccgcccccggtgcgccccaccccttccacttgcacgggcacgcgttcgcggtcgtccgcagcgccggcagcacggtttacaactacgacaaccccatcttccgcgacgtcgtcagcacggggacgcctgcggccggtgacaacgtcaccatccgcttccgcaccgacaaccccggcccgtggttcctccactgccacatcgacttccacctcgaggccggcttcgccgtcgtgttcgcggaggacatccccgacgtcgcgtcggcgaaccccgtcccccaggcgtggtccgacctctgcccgacctacgacgcgctcgacccgagcgaccagtag

SEQ ID NO: 2 - protein, 520 aa, Polyporus pinsitus
MSRFHSLLAFVVASLTAVAHAGIGPVADLTITNAAVSPDGFSRQAVVVNGGTPGPLITGNMGDRFQLNVIDNLTNHTMVKSTSIHWHGFFQKGTNWADGPAFINQCPISSGHSFLYDFQVPDQAGTFWYHSHLSTQYCDGLRGPFVVYDPNDPAADLYDVDNDDTVITLVDWYHVAAKLGPAFPLGADATLINGKGRSPSTTTADLSVISVTPGKRYRFRLVSLSCDPNYTFSIDGHNMTIIETDSINTAPLVVDSIQIFAAQRYSFVLEANQAVDNYWIRANPNFGNVGFTGGINSAILRYDGAAAVEPTTTQTTSTAPLNEVNLHPLVTTAVPGSPVAGGVDLAINMAFNFNGTNFFINGTSFTPPTVPVLLQIISGAQNAQDLLPSGSVYSLPSNADIEISFPATAAAPGAPHPFHLHGHAFAVVRSAGSTVYNYDNPIFRDVVSTGTPAAGDNVTIRFRTDNPGPWFLHCHIDFHLEAGFAVVFAEDIPDVASANPVPQAWSDLCPTYDALDPSDQ

SEQ ID NO: 3 - DNA, 1563 bp, Trametes versicolor
atgtcgaggtttcactctcttctcgctttcgtcgttgcttcccttacggctgtggcccacgctggtatcggtcccgtcgccgacctaaccatcaccaacgcagcggtcagccccgacgggttttctcgccaggccgtcgtcgtgaacggcggcacccctggccctctcatcaccggtaacatgggggatcgcttccagctcaatgtcatcgacaacctcaccaaccacacgatgctgaagagcacgagtattcactggcacggtttcttccagaagggcaccaactgggccgacggtcccgccttcatcaaccagtgcccgatctcatctggtcactcgttcctgtacgacttccaggttcctgaccaggctggtaccttctggtatcacagtcacttgtctacgcagtactgtgatggtttgaggggtccgttcgttgtttacgacccgaatgacccggccgccgacctgtacgacgtcgacaacgacgacactgtcattacccttgtggattggtaccacgtcgccgcgaagctgggccccgcattccctctcggcgccgacgccaccctcatcaacggtaagggacgctcccccagcacgaccaccgcggacctctcagttatcagcgtcaccccgggtaaacgctaccgtttccgcctggtgtccctgtcgtgcgaccccaactacacgttcagcatcgatggtcacaacatgacgatcatcgagaccgactcaatcaacacggcgcccctcgtcgtcgactccattcagatcttcgccgcccagcgttactccttcgtgctcgaggccaaccaggccgtcgacaactactggattcgcgccaacccgaacttcggtaacgtcgggttcaccggcggcattaactcggctatcctccgctacgatggtgccgctgccgtggagcccaccaccacgcaaaccacgtcgtctgcgccgctcaacgaggtcaacctgcacccgctggttgccaccgctgtgcctggctcgcccgtcgctggtggtgtcgacctggccatcaacatggcgttcaacttcaacggcaccaacttcttcatcaacggcgcgtctttcacgcccccgaccgtgcctgtcctcctccagatcatcagcggcgcgcagaacgcgcaggacctcctgccctccggcagcgtctactcgcttccctcgaacgccgacatcgagatctccttccccgcgaccgccgccgcccccggtgcgccccaccccttccacttgcacgggcacgcgttcgcggtcgtccgcagcgccggcagcacggtctacaactacgacaaccccatcttccgcgacgtcgtcagcacggggacgcctgcggccggtgacaacgtcaccatccgcttccgcaccgacaaccccggcccgtggttcctccactgccacatcgacttccacctcgaggccggcttcgccgtcgtgttcgcggaggacatccccgacgtcgcgtcggcgaaccctgtcccccaggcgtggtccgacctctgcccgacctacgacgcgctcgacccgagcgaccagtag

SEQ ID NO: 4 - protein, 520 aa, Trametes versicolor
MSRFHSLLAFVVASLTAVAHAGIGPVADLTITNAAVSPDGFSRQAVVVNGGTPGPLITGNMGDRFQLNVIDNLTNHTMLKSTSIHWHGFFQKGTNWADGPAFINQCPISSGHSFLYDFQVPDQAGTFWYHSHLSTQYCDGLRGPFVVYDPNDPAADLYDVDNDDTVITLVDWYHVAAKLGPAFPLGADATLINGKGRSPSTTTADLSVISVTPGKRYRFRLVSLSCDPNYTFSIDGHNMTIIETDSINTAPLVVDSIQIFAAQRYSFVLEANQAVDNYWIRANPNFGNVGFTGGINSAILRYDGAAAVEPTTTQTTSSAPLNEVNLHPLVATAVPGSPVAGGVDLAINMAFNFNGTNFFINGASFTPPTVPVLLQIISGAQNAQDLLPSGSVYSLPSNADIEISFPATAAAPGAPHPFHLHGHAFAVVRSAGSTVYNYDNPIFRDVVSTGTPAAGDNVTIRFRTDNPGPWFLHCHIDFHLEAGFAVVFAEDIPDVASANPVPQAWSDLCPTYDALDPSDQ

SEQ ID NO: 5 - DNA, 1563 bp, Trametes versicolor
  misc_feature (1119)..(1119): n is a, c, g, or t
  misc_feature (1251)..(1251): n is a, c, g, or t
  misc_feature (1305)..(1305): n is a, c, g, or t
atgtcgaggtttcactctcttttcgctttcgtcgttgcttcccttacggctgtggcccacgctggtatcggtcccgtcgccgacctaaccatcaccaacgcagcggtcagccccgacgggttttctcgccaggccgtcgtcgtgaacggcggcacccctggccctctcatcacgggtaacatgggggatcgcttccagctcaatgtcatcgacaaccttaccaaccacacgatgctgaagagcacgagtattcactggcacggtttcttccagaagggcaccaactgggccgacggtcccgccttcatcaaccagtgcccgatctcatctggtcactcgttcctgtacgacttccaggttcctgaccaggctggtaccttctggtatcacagtcacttgtctacgcagtactgtgatggtttgaggggtccgttcgttgtttacgacccgaacgacccggccgccgacctgtacgacgtcgacaacgacgacactgtcattacccttgtggattggtaccacgtcgccgcgaagctgggccccgcattccctctcggcgccgacgccaccctcatcaacggtaagggacgctcccccagcacgaccaccgcggacctctcagttatcagtgtcaccccgggtaaacgctaccgtttccgcctggtgtccctgtcgtgcgaccccaactacacgttcagcatcgatggtcacaacatgacgatcatcgagaccgactcaatcaacacggcgcccctcgtcgtcgactccattcagattttcgccgcccagcgttactccttcgtgctcgaggccaaccaggccgtcgacaactactggattcgcgccaacccaaacttcggtaacgtcgggtttaccggcggcattaactcggctatcctccgctacgatggtgccgctgccgtggagcccaccaccacgcaaaccacctcgactgcgccgctcaacgaggtcaacctgcacccgctggttgccaccgctgtgcctggctcgcccgtcgctggtggtgtcgacctggccatcaacatggcgttcaacttcaacggcaccaacttcttcatcaacggcgcgtctttcacgcccccgaccgtgcctgtcctncttcagatcatcagcggcgcgcagaacgcgcaggacctcctgccctccggcagcgtctactcgcttccctcgaacgccgacatcgagatctccttcccggcgaccgccgccgcccccggtgcgccccacccnttccacttgcacgggcacgcgttcgcggtcgtccgcagcgccggcagcacggtntacaactacgacaaccccatcttccgcgacgtcgtcagcacggggacgcctgcggccggtgacaatgtcaccatccgcttccgcaccgacaaccccggcccgtggttcctccactgccacatcgacttccacctcgaggccggcttcgccgtcgtgttcgcggaggacatccccgacgtcgcgtcggcgaaccccgtcccccaggcgtggtccgacctctgcccgacctacgacgcgcgcgacccgagcgaccagtaa

SEQ ID NO: 6 - protein, 520 aa, Trametes versicolor
MSRFHSLFAFVVASLTAVAHAGIGPVADLTITNAAVSPDGFSRQAVVVNGGTPGPLITGNMGDRFQLNVIDNLTNHTMLKSTSIHWHGFFQKGTNWADGPAFINQCPISSGHSFLYDFQVPDQAGTFWYHSHLSTQYCDGLRGPFVVYDPNDPAADLYDVDNDDTVITLVDWYHVAAKLGPAFPLGADATLINGKGRSPSTTTADLSVISVTPGKRYRFRLVSLSCDPNYTFSIDGHNMTIIETDSINTAPLVVDSIQIFAAQRYSFVLEANQAVDNYWIRANPNFGNVGFTGGINSAILRYDGAAAVEPTTTQTTSTAPLNEVNLHPLVATAVPGSPVAGGVDLAINMAFNFNGTNFFINGASFTPPTVPVLLQIISGAQNAQDLLPSGSVYSLPSNADIEISFPATAAAPGAPHPFHLHGHAFAVVRSAGSTVYNYDNPIFRDVVSTGTPAAGDNVTIRFRTDNPGPWFLHCHIDFHLEAGFAVVFAEDIPDVASANPVPQAWSDLCPTYDARDPSDQ

SEQ ID NO: 7 - DNA, 1563 bp, Trametes versicolor
atgtcgaggtttcactctcttctcgctttcgtcgttgcttcccttacggctgtggcccacgctggtatcggtcccgtcgccgacctcaccatcaccaacgcagcggtcagccctgatgggttttctcgccaggccgtcgtcgtgaacggcggcacccctggccctctcatcaccggtaacatgggggatcgcttccagctcaatgtcatcgacaacctcaccaaccacacgatgctgaagagcaccagtattcactggcacggtttcttccagaagggcacgaactgggccgacggtcccgccttcatcaaccagtgcccgatctcatctggtcactcgttcctgtacgacttccaggttcctgaccaggctggcaccttctggtaccacagtcacttgtccacgcagtactgtgatggtctgaggggtccgttcgttgtttacgacccgaatgacccggccgccgacttgtacgacgtcgacaacgacgacactgtcattaccctcgtggattggtaccacgtcgccgcgaacgtgggccctgccttccctctcggcgccgatgcgaccctcatcaatggcaagggacgctcccccagcacgaccaccgcggacctctctgttatcagcgtcaccccgggtaaacgctaccgtttccgcctggtgtccctgtcgtgcgaccccaactacacgttcagcatcgatggtcacaacatgacgatcatcgagaccgactcgatcaacacggcgcccctcgtggtcgactccattcagatcttcgccgcccagcgttactccttcgtgctcgaggccaaccaggccgtcgacaactactggattcgcgccaaccccaacttcggtaacgtcgggttcaccggcggcatcaactcggctatcctccgctacgatggtgccgctgccgtcgagcccactaccacgcagaccacttcgaccgagccgctcaatgaggtcaacctgcacccgctggttgccaccgctgtgcctggctctcccgttgcgggtggtgtcgacctggccatcaacatggcgttcaacttcaacggcaccaacttcttcatcaacggcgcgtctttcacgcccccgaccgtgcctgtcctcctccagatcatcagcggcgcgcagaacgcgcaagacctcctgccctctggcagcgtctactcgctcccctcgaacgccgacatcgagatctcgttccccgccaccgccgccgcccctggtgcgccccaccccttccacttgcacgggcacgcgttcgcggtcgtccgcagcgccggcagcacagtctacaactacgacaaccccatcttccgcgacgtcgtcagcacggggacgcctgcggccggtgacaacgtcaccatccgcttccgcaccgacaaccccggcccgtggttcctccattgccacatcgacttccacctcgaggccggtttcgccgtcgtgttcgcggaggacatccccgacgttgcgtcggcgaaccccgtgccccaggcgtggtccgacctctgcccgacctacgatgcgctcgacccgagcgaccagtaa

SEQ ID NO: 8 - protein, 520 aa, Trametes versicolor
MSRFHSLLAFVVASLTAVAHAGIGPVADLTITNAAVSPDGFSRQAVVVNGGTPGPLITGNMGDRFQLNVIDNLTNHTMLKSTSIHWHGFFQKGTNWADGPAFINQCPISSGHSFLYDFQVPDQAGTFWYHSHLSTQYCDGLRGPFVVYDPNDPAADLYDVDNDDTVITLVDWYHVAANVGPAFPLGADATLINGKGRSPSTTTADLSVISVTPGKRYRFRLVSLSCDPNYTFSIDGHNMTIIETDSINTAPLVVDSIQIFAAQRYSFVLEANQAVDNYWIRANPNFGNVGFTGGINSAILRYDGAAAVEPTTTQTTSTEPLNEVNLHPLVATAVPGSPVAGGVDLAINMAFNFNGTNFFINGASFTPPTVPVLLQIISGAQNAQDLLPSGSVYSLPSNADIEISFPATAAAPGAPHPFHLHGHAFAVVRSAGSTVYNYDNPIFRDVVSTGTPAAGDNVTIRFRTDNPGPWFLHCHIDFHLEAGFAVVFAEDIPDVASANPVPQAWSDLCPTYDALDPSDQ

SEQ ID NO: 9 - DNA, 1563 bp, Trametes sp.
atgtcgaggtttcactctcttctcgctttcgtcgttgcttcccttacggctgtggcccacgctggtattggtcccgtcgccgacctcaccatcaccaacgcagcggtcagccccgacgggttttctcgccaggccgtcgtcgtgaacggcggcacccctggccctctcatcacgggtaacatgggggatcgcttccagctcaatgtcatcgacaaccttaccaaccacacgatgctgaagagcacgagtattcactggcacggtttcttccagaagggcaccaactgggccgacggtcccgccttcatcaaccagtgcccgatctcatctggtcactcgttcctgtacgacttccaggttcctgaccaggctggtaccttctggtatcacagtcacttgtccacgcagtactgtgatggtctgaggggtccgttcgttgtttacgacccgaatgatccggccgccgacctgtacgacgtcgacaacgacgacactgtcattacccttgtggattggtaccacgtcgccgcgaagctgggccccgcattccctctcggcgccgacgccaccctcatcaacggtaagggacgctcccccagcacgaccaccgcggacctctcagttatcagcgtcaccccgggtaaacgctaccgtttccgcctggtctccctgtcgtgcgaccccaactacacgttcagcatcgatggtcacaacatgacgatcatcgagaccgactcaatcaacacggcgcccctcgtcgtcgactccattcagatcttcgccgcccagcgttactccttcgtgctcgaggccaaccaggccgtcgacaactactggattcgtgcaaacccgagcttcggtaatgtcgggttcacgggtggcatcaactcggctatcctccgctacgatggtgccgctgccatcgagcccaccaccacgcagaccacttcgacggagccgctcaacgaggtgaacctgcacccgctggtcgccaccgctgtgcccggctcccccgttgcgggtggtgtcgacctggccatcaacatggcgttcaacttcaacggcaccaacttcttcatcaacggggcgtctttcacgcccccgactgtgcctgtcctgctccagatcatcagcggcgcacagaacgcgcaagacctcctgccctccggcagcgtctactcgctcccctcgaacgctgacattgagatctccttccccgccaccaccgccgcccccggcgcgccccaccccttccacttgcacgggcacgcgttcgcggtcgtccgcagcgccggcagcacggtctacaactacgacaaccccatcttccgcgacgtcgtcagcacggggacgcctgcggccggtgacaacgtcaccatccgcttccgcaccgacaaccccggcccgtggttcctccactgccacatcgacttccacctcgaggccggcttcgccgtcgtgttcgcggaggacatccccgacgtcgcgtcggcgaaccccgtcccccaggcgtggtccgacctctgcccgacctacgacgcgctcgacccgagcgaccagtaa

SEQ ID NO: 10 - protein, 520 aa, Trametes sp.
MSRFHSLLAFVVASLTAVAHAGIGPVADLTITNAAVSPDGFSRQAVVVNGGTPGPLITGNMGDRFQLNVIDNLTNHTMLKSTSIHWHGFFQKGTNWADGPAFINQCPISSGHSFLYDFQVPDQAGTFWYHSHLSTQYCDGLRGPFVVYDPNDPAADLYDVDNDDTVITLVDWYHVAAKLGPAFPLGADATLINGKGRSPSTTTADLSVISVTPGKRYRFRLVSLSCDPNYTFSIDGHNMTIIETDSINTAPLVVDSIQIFAAQRYSFVLEANQAVDNYWIRANPSFGNVGFTGGINSAILRYDGAAAIEPTTTQTTSTEPLNEVNLHPLVATAVPGSPVAGGVDLAINMAFNFNGTNFFINGASFTPPTVPVLLQIISGAQNAQDLLPSGSVYSLPSNADIEISFPATTAAPGAPHPFHLHGHAFAVVRSAGSTVYNYDNPIFRDVVSTGTPAAGDNVTIRFRTDNPGPWFLHCHIDFHLEAGFAVVFAEDIPDVASANPVPQAWSDLCPTYDALDPSDQ

SEQ ID NO: 11 - DNA, 1563 bp, Trametes versicolor
atgtcgaggtttcactctcttctcgctttcgtcgttgcttcccttgcggctgtggcccacgctggtatcggtcctgtcgccgacctcaccatcaccaacgcagcggtcagccccgacgggttttctcgccaggccgtcgtcgtgaacggcggcacccctggccctctcatcaccggtaacatgggggatcgcttccagctcaatgtcatcgacaacctcacgaaccacacgatgctgaagagcaccagtattcactggcacggtttcttccagaagggcaccaactgggccgacggtcccgccttcatcaaccagtgcccgatctcatctggccactcgttcctgtatgacttccaggttcctgaccaggctggcaccttctggtaccacagtcacttgtccacgcagtactgtgatggtctgaggggtccattcgttgtttacgacccgaatgacccggccgccgacctgtacgacgtcgacaacgacgacacggtcattacccttgcggattggtaccacgtcgccgcgaagctgggccccgcattccctctcggcgccgacgccactctcatcaacggtaagggacgctcccccagcacgaccaccgcggacctcactgttatcagcgtcactccgggtaaacgttaccgtttccgcctggtgtccctgtcgtgcgaccccaaccacaccttcagcatcgatggccacaacatgacgatcatcgagaccgactcgatcaacacggcgcccctcgtggtcgactccattcagatcttcgccgcccagcgttactccttcgtgctcgaggccaaccaggccgtcgacaactactggattcgcgccaacccgagcttcggtaacgtcgggttcaccggcggcatcaactcggctatccttcgctatgatggcgccgctgccatcgagcccaccaccacgcagaccacttcgaccgagccgctcaacgaggtcaacctgcacccgctggttgccaccgctgtccctggctctcccgttgcgggtggtgttgacctggccatcaatatggcgttcaacttcaatggcaccaacttcttcatcaacggcgcgtctttcacgcccccgaccgtgcctgtcctcctccagatcatcagcggcgcgcagaacgcgcaggacctcctgccctccggcagcgtatactcgctcccctcgaacgccgacatcgagatctccttccccgccaccgccgctgcccccggtgcgccccaccccttccacttgcatgggcacgcgttcgcggtcgtccgcagcgccggcagcacggtctacaactacgacaaccccatcttccgcgacgtcgtcagcacggggacgcctgcggccggtgacaacgtcaccatccgcttccgcaccgacaaccccggcccgtggttcctccactgccacatcgacttccacctcgaggccggcttcgccgtcgtgttcgcggaggacatccccgacgtcgcgtcggcgaaccccgtcccccaggcgtggtccgacctctgcccgacctacgacgcgctcgaccccagcgaccagtaa

SEQ ID NO: 12 - protein, 520 aa, Trametes versicolor
MSRFHSLLAFVVASLAAVAHAGIGPVADLTITNAAVSPDGFSRQAVVVNGGTPGPLITGNMGDRFQLNVIDNLTNHTMLKSTSIHWHGFFQKGTNWADGPAFINQCPISSGHSFLYDFQVPDQAGTFWYHSHLSTQYCDGLRGPFVVYDPNDPAADLYDVDNDDTVITLADWYHVAAKLGPAFPLGADATLINGKGRSPSTTTADLTVISVTPGKRYRFRLVSLSCDPNHTFSIDGHNMTIIETDSINTAPLVVDSIQIFAAQRYSFVLEANQAVDNYWIRANPSFGNVGFTGGINSAILRYDGAAAIEPTTTQTTSTEPLNEVNLHPLVATAVPGSPVAGGVDLAINMAFNFNGTNFFINGASFTPPTVPVLLQIISGAQNAQDLLPSGSVYSLPSNADIEISFPATAAAPGAPHPFHLHGHAFAVVRSAGSTVYNYDNPIFRDVVSTGTPAAGDNVTIRFRTDNPGPWFLHCHIDFHLEAGFAVVFAEDIPDVASANPVPQAWSDLCPTYDALDPSDQ

SEQ ID NO: 13 - DNA, 1563 bp, Trametes versicolor
atgtcgaggtttcactctcttctcgctttcgtcgttgcttcccttgcggctgtggcccacgctggtatcggtcctgtcgccgacctcaccatcaccaacgcagcggtcagccccgacgggttttctcgccaggccgtcgtcgtgaacggtggcacccctggccctctcatcaccggtaacatgggggatcgcttccagctcaatgtcatcgacaacctcacggaccacacgatgctgaagagcaccagtattcactggcacggtttcttccagaagggcaccaactgggccgacggtcccgccttcatcaaccagtgcccgatctcatctggccactcgttcctgtatgacttccaggttcctgaccaggctggcaccttctggtaccacagtcacttgtccacgcagtactgtgatggtctgaggggtccgttcgttgtttacgacccgaatgacccggccgccgacctgtacgacgtcgacaacgacgacacggtcattacccttgcggattggtaccacgtcgccgcgaagctgggccccgcattccctctcggcgccgacgccactctcatcaacggtaagggacgctcccccagcacgaccaccgcggacctcactgttatcagcgtcactccgggtaaacgttaccgtttccgcctggtgtccctgtcgtgcgaccccaaccacaccttcagcatcgatggccacaacatgacgatcatcgagaccgactcgatcaacacggcgcccctcgtggtcgactccattcagatcttcgctgcccagcgttactccttcgtgctcgaggccaaccaggccgtcgacaactactggattcgcgccaacccgagcttcggtaacgtcgggttcaccggcggcatcaactcggctatcctccgctatgatggcgccgctgccatcgagcccaccaccacgcagaccacttcgaccgagccgctcaacgaggtcaacctgcacccgctggttgccaccgctgtccctggctctcccgctgcgggtggtgttgacctggccatcaatatggcgttcaacttcaatggcaccaacttcttcatcaacggcgcgtctttcacgcccccgaccgtgcctgtcctcctccagatcatcagcggcgcgcagaacgcgcaggacctcctgccctccggcagcgtatactcgctcccctcgaacgccgacatcgagatctccttccccgccaccgccgctgcccccggtgcgccccaccccttccacttgcacgggcacgcgttcgcggtcgtccgcagcgccggcagcacggtctacaactacgacaaccccatcttccgcgacgtcgtcagcacggggacgcctgcggccggtgacaacgtcaccatccgcttccgcaccgacaaccccggcccgtggtttctccactgccacatcgacttccacctcgaggccggcttcgccgtcgtgtttgcggaggacatccccgatgtcgcatcggcgaaccccgtcccccaggcgtggtccgacctctgcccgacctacgacgcgcgcgacccgagcgaccagtaa

SEQ ID NO: 14 - protein, 520 aa, Trametes versicolor
MSRFHSLLAFVVASLAAVAHAGIGPVADLTITNAAVSPDGFSRQAVVVNGGTPGPLITGNMGDRFQLNVIDNLTDHTMLKSTSIHWHGFFQKGTNWADGPAFINQCPISSGHSFLYDFQVPDQAGTFWYHSHLSTQYCDGLRGPFVVYDPNDPAADLYDVDNDDTVITLADWYHVAAKLGPAFPLGADATLINGKGRSPSTTTADLTVISVTPGKRYRFRLVSLSCDPNHTFSIDGHNMTIIETDSINTAPLVVDSIQIFAAQRYSFVLEANQAVDNYWIRANPSFGNVGFTGGINSAILRYDGAAAIEPTTTQTTSTEPLNEVNLHPLVATAVPGSPAAGGVDLAINMAFNFNGTNFFINGASFTPPTVPVLLQIISGAQNAQDLLPSGSVYSLPSNADIEISFPATAAAPGAPHPFHLHGHAFAVVRSAGSTVYNYDNPIFRDVVSTGTPAAGDNVTIRFRTDNPGPWFLHCHIDFHLEAGFAVVFAEDIPDVASANPVPQAWSDLCPTYDARDPSDQ

SEQ ID NO: 15 - DNA, 1563 bp, Trametes pubescens
atgtcgaggttccaatctcttctcgctttcgtcgttgcttctcttgcggctgtggcccacgcaggtatcggtcctgtcgccgacctcaccatctccaatgctgccgtcagccccgacggcttttctcgccaggccgttgtggtgaacgggggcacccctggtcccctcatcaccggtaacaagggggacaacttccagctcaatgtcatcgacaacctgacgaaccacacgatgctgaagagcaccagtatccactggcacggtttcttccagaagggcacgaactgggccgacggtcccgccttcatcaaccagtgccctatctcatctggcaactcgttcctgtacaacttccaggtgcctgaccaggctggcaccttttggtaccacagtcacttgtccacgcagtactgtgacggtctgagggggccgttcgttgtctacgacccgaatgacccgagcgctgacttgtacgacgttgacaacgacgacaccgtcatcacgctcgtggattggtaccacgtcgcggcgaagctaggccccgccttccctctcggcgccgacgccaccctcatcaatggtaaggggcgctcccccagtacgacgacggcggacctcgctgttatcagcgtcactgcgggtaaacgctaccgcttccgcctggtgtccctgtcgtgcgaccccaactacgtcttcagcatcgatggtcacaacatgacgatcatcgagaccgactcgatcaacacgcagccccttgtggtcgactccattcagatctttgccgcccagcgatactctttcgtgctggaggctaaccaggcggtcgacaactactggattcgtgccaacccgaacttcggaaacgtcgggttcaccggcggtatcaactcggctattctccgctacgatggcgccgccgccattgagcccacgaccacgcagaccacttcgacgcagcccctcaacgaggtgaacctgcaccctcttgtggccaccgctgtgcccggctctcccgttgcgggtggcgtcgacctagccatcaacatggcgttcaacttcaacggcaccaacttcttcatcaacggcgcatccttcacgcccccgaccgtgcctgtcctgctccagatcatcagcggtgcgcagaacgcgcaggacctcctcccgtccggcagcgtctactcgctcccctcgaacgcggacatcgaaatctcgttccccgccaccaccgccgcgcccggtgctccccaccccttccacttgcacgggcacgcgttcgcggtcgtccgcagcgccggcagcaccgtctacaactacgacaacccgatcttccgcgacgtcgtcagcacggggacgcctgcggccggtgacaacgtcacgatccgcttccgcaccgacaaccccggcccgtggttcctccactgccacatcgacttccaccttgaggccggcttcgccgtcgtgttcgcggaggatatccctgacgtcgcgtcggcgaacccggtcccccaggcgtggtctgacctctgccccatctacgacgcgctcgaccccagcgaccagtag

SEQ ID NO: 16 - protein, 520 aa, Trametes pubescens
MSRFQSLLAFVVASLAAVAHAGIGPVADLTISNAAVSPDGFSRQAVVVNGGTPGPLITGNKGDNFQLNVIDNLTNHTMLKSTSIHWHGFFQKGTNWADGPAFINQCPISSGNSFLYNFQVPDQAGTFWYHSHLSTQYCDGLRGPFVVYDPNDPSADLYDVDNDDTVITLVDWYHVAAKLGPAFPLGADATLINGKGRSPSTTTADLAVISVTAGKRYRFRLVSLSCDPNYVFSIDGHNMTIIETDSINTQPLVVDSIQIFAAQRYSFVLEANQAVDNYWIRANPNFGNVGFTGGINSAILRYDGAAAIEPTTTQTTSTQPLNEVNLHPLVATAVPGSPVAGGVDLAINMAFNFNGTNFFINGASFTPPTVPVLLQIISGAQNAQDLLPSGSVYSLPSNADIEISFPATTAAPGAPHPFHLHGHAFAVVRSAGSTVYNYDNPIFRDVVSTGTPAAGDNVTIRFRTDNPGPWFLHCHIDFHLEAGFAVVFAEDIPDVASANPVPQAWSDLCPIYDALDPSDQ

SEQ ID NO: 17 - DNA, 1563 bp, Trametes hirsuta
atgtcgaggttccagtctctgctcgccttcgtcgtcgcctctctcgcggctgtggcccatgccgccattgggcccaccgctgacctcaccatctccaatgccgaggtcagccccgatgggttcgctcgtcaggctgtggttgtcaacaatgttaccccgggacccctcgtcgcgggcaacaagggtgaccgcttccaactcaatgtcatcgacaacctcacgaaccacactatgctgaagagcacgagtatccactggcatggcttcttccagaaggggacaaactgggctgatggtcccgcgtttgtgaaccagtgccctatttcctctgggcactcgttcctctacgatttccaggttcctgaccaggccggtaccttctggtaccacagccacttgtccactcagtactgtgacggcctgcggggtcctttcgtcgtgtacgatcccaatgacccgcacgcgagtttgtatgacgtcgacaatgacgacaccgtgatcaccctcgcggattggtaccacactgccgcgaagctcggccccgcgttcccactgggtgcggatgctacccttatcaacgggctcgggcgttcccccagcaccacggcggcggacctcgcagtcatcaacgtcacgaagggcaaacgctaccgtttccgcctggtctccctgtcgtgtgaccccaaccacacgttcagcatcgatggtcatgacttgacgatcatcgaggtggactccatcaactcgcaacctctggtggttgactccatccagattttcgctgcgcagcggtactcctttgtgttgaatgccgaccaggatgtcggtaactactggattcgcgccaaccccaacttcggcaacgtcggatttgcgggtggtatcaactcggccatcctgcgctacgacggcgccgacccggttgagcccaccacgactcagactacgccgaccaagcccctgaacgaggtcgacttgcacccgctcgccaccatggctgtgcccggttccccagtcgccggtggtgttgacacggctatcaacatggccttcaacttcaatggtaccaacttcttcatcaacggcgcgagctttgtgccccccaccgtgccggtcctgctccagatcatcagcggcgcccagaacgcccaggatctcctcccgtctggcagcgtctactccctcccgtcaaacgcggatatcgagatctcgttccctgctacggcggctgctccgggtgcccctcaccccttccacttgcacggtcacgccttcgccgtcgtccgtagcgctggcagcaccgtctacaactacgacaaccccatcttccgcgacgtcgtcagcacggggacgcctgcggccggtgacaacgtcaccatccgcttccgcaccgacaaccctggcccgtggttcctccactgccacatcgacttccaccttgaggccggctttgcggtcgtgttcgcggaggacatccccgacgtcgcgtcggcgaaccccgtccctcaggcatggtctgatctgtgccccatctatgacgcactcgatgtcaacgaccagtag

SEQ ID NO: 18 - protein, 520 aa, Trametes hirsuta
MSRFQSLLAFVVASLAAVAHAAIGPTADLTISNAEVSPDGFARQAVVVNNVTPGPLVAGNKGDRFQLNVIDNLTNHTMLKSTSIHWHGFFQKGTNWADGPAFVNQCPISSGHSFLYDFQVPDQAGTFWYHSHLSTQYCDGLRGPFVVYDPNDPHASLYDVDNDDTVITLADWYHTAAKLGPAFPLGADATLINGLGRSPSTTAADLAVINVTKGKRYRFRLVSLSCDPNHTFSIDGHDLTIIEVDSINSQPLVVDSIQIFAAQRYSFVLNADQDVGNYWIRANPNFGNVGFAGGINSAILRYDGADPVEPTTTQTTPTKPLNEVDLHPLATMAVPGSPVAGGVDTAINMAFNFNGTNFFINGASFVPPTVPVLLQIISGAQNAQDLLPSGSVYSLPSNADIEISFPATAAAPGAPHPFHLHGHAFAVVRSAGSTVYNYDNPIFRDVVSTGTPAAGDNVTIRFRTDNPGPWFLHCHIDFHLEAGFAVVFAEDIPDVASANPVPQAWSDLCPIYDALDVNDQ

SEQ ID NO: 19 - DNA, 1563 bp, Trametes hirsuta
atgtcgaggttccagtctctgctcgccttcgtcgtcgcctccctcgcggctgtggcccatgccgccattgggcccaccgctgacctcaccatctccaatgccgaggtcagccccgatgggttcgctcgtcaggctgtggttgtcaacaatgttaccccgggacccctagtcgcgggcaacaagggtgaccgcttccaactcaatgtcatcgacaacctcacgaaccacactatgctgaagagcacgagtatccactggcatggcttcttccagaaggggacaaactgggctgatggtcccgcgtttgtgaaccagtgccctatttcctctgggcactcgttcctctacgatttccaggttcctgaccaggccggtaccttctggtaccacagccacttgtccactcagtactgtgacggcctgcggggtcctttcgtcgtgtacgatcccaatgacccgcacgcgagcttgtatgacgtcgacaatgacgacaccgtgatcaccctcgcggattggtaccacactgccgcgaagctcggccccgccttcccactgggtgcggatgctacccttatcaacgggctcgggcgttcccccagcaccacggcggcggacctcgcggtcatcaacgtcacgaagggcaaacgctaccgtttccgcctggtctccctgtcgtgtgaccccaaccacacgttcagcatcgatggtcatgacttgacgatcatcgaggtggactccatcaactcccaacctctggtggttgactccatccagattttcgctgcgcagcggtactcctttgtgttgaatgccgaccaggacgtcggtaactactggattcgcgccaaccccaacttcggcaacgtcggatttgcgggtggtatcaactcggccatcctgcgctacgacggcgccgacccggttgagcccaccacgactcagactacgccgaccaagcccctgaacgaggtcgacttgcacccgctcgccaccatggctgtgcccggttccccagtcgccggtggtgttgacacggctatcaacatggccttcaacttcaatggtaccaacttcttcatcaacggcgcgagctttgtgccccccaccgtgccggtcctgctccagatcatcaggcgcgcccagaacgcccaggatctcctcccgtctggcagcgtctactccctcccgtcgaacgcggacatcgagatctcgttccctgctaccgcggcccctccgggtgcccctcaccccttccacttgcatggtcacgccttcgccgttgtccgtagcgctggcagcaccgtctacaactacgacaaccccatcttccgcgacgtcgtcagcacggggacgcctgcggccggtgacaacgtcaccatccgcttccgcaccgacaaccccggcccgtggttcctccactgccacatcgacttccaccttgaggccggctttgcggtcgtgttcgctgaggacatccccgacgtcgcgtcggcgaaccctgtccctcaggcgtggtctgatctgtgccccatctatgacgcactcgatgtcaacgaccagtag

SEQ ID NO: 20 - protein, 520 aa, Trametes hirsuta
MSRFQSLLAFVVASLAAVAHAAIGPTADLTISNAEVSPDGFARQAVVVNNVTPGPLVAGNKGDRFQLNVIDNLTNHTMLKSTSIHWHGFFQKGTNWADGPAFVNQCPISSGHSFLYDFQVPDQAGTFWYHSHLSTQYCDGLRGPFVVYDPNDPHASLYDVDNDDTVITLADWYHTAAKLGPAFPLGADATLINGLGRSPSTTAADLAVINVTKGKRYRFRLVSLSCDPNHTFSIDGHDLTIIEVDSINSQPLVVDSIQIFAAQRYSFVLNADQDVGNYWIRANPNFGNVGFAGGINSAILRYDGADPVEPTTTQTTPTKPLNEVDLHPLATMAVPGSPVAGGVDTAINMAFNFNGTNFFINGASFVPPTVPVLLQIIRRAQNAQDLLPSGSVYSLPSNADIEISFPATAAPPGAPHPFHLHGHAFAVVRSAGSTVYNYDNPIFRDVVSTGTPAAGDNVTIRFRTDNPGPWFLHCHIDFHLEAGFAVVFAEDIPDVASANPVPQAWSDLCPIYDALDVNDQ

SEQ ID NO: 21 - DNA, 1563 bp, Trametes sp.
atgtcgaggttccagtctctgctcgccttcgtcgtcgcctccctcgcggctgttgctcatgccgccattgggcccaccgctgacctcaccatctctaatgccgaggtcagccccgatgggttcgctcgtcaggccgtggttgtcaacaacgttaccccggggcccctggtcgcgggtaacaagggtgaccgcttccaactcaatgtcatcgacaacctcaccaaccacaccatgctgaagagcacgagtattcactggcacggcttcttccagaaggggacgaactgggctgatggtcctgcgttcgtgaaccagtgccctatctcgtctgggcattcgttcctgtacgacttccaggttccggatcaggccggcacattctggtaccacagtcacctgtccacgcagtactgcgacggcctgcgcggtcccttcgttgtgtacgatccgaatgacacgcacgcgagcttgtatgacgtcgacaacgacgacaccgtgatcacactcgcggattggtaccacaccgccgcaaagctcggaccaacatttccactgggtgccgacgcaacgctgatcaacgggcttggccgctccccgagcaccacggctgcggacctcgcagtcatcaacgtcacgaaggggaaacgctaccgtttccgcctcgtctccctgtcgtgtgatcccaaccacacgttcagcatcgatggtcatgacttgacgatcatcgaagtggactccatcaactcccagcctctggtggttgactccatccagatcttcgctgcgcagcggtactccttcgtgttgaatgccgaccaggatgtcggcaactactggatccgtgccaaccctagcttcggaaacgtcggatttgcgggcggtatcaactcggccatcctgcgctacgacggcgccgacccggtcgagcccaccacgacgcagactacgcccactaagcccctcaacgaggttgacctgcacccactcgacaccatggctgtgcccggctccccggtcgccggtggtgttgacaaggctatcaacatggccttcaacttcaacggtaccaacttcttcatcaacggcgcaagctttgtgccccctaccgtgccggtcctgcttcagatcatcagcggcgctcaaaacgcccaggatcttctcccctctggcagtgtctactcgctcccggcgaacgctgacatcgagatctcgttccctgctaccgcggctgctccgggtgcccctcatcccttccacttgcacggtcacgccttcgccgtcgttcgcagcgctggcagcaccgtgtacaactacgacaaccccatcttccgcgacgtcgtcagcacggggacgcctgcggccggtgacaacgtcaccatccgcttccgcaccgacaaccctggcccgtggttcctccactgccacatcgacttccacctcgaggccggttttgcggtcgtgatggcggaggacattcctgacgtcgcgtcagcgaaccctgtcccccaggcgtggtctgacctgtgccccatctacgacgcgctcgatgtcaacgaccagtag

SEQ ID NO: 22 - protein, 520 aa, Trametes sp.
MSRFQSLLAFVVASLAAVAHAAIGPTADLTISNAEVSPDGFARQAVVVNNVTPGPLVAGNKGDRFQLNVIDNLTNHTMLKSTSIHWHGFFQKGTNWADGPAFVNQCPISSGHSFLYDFQVPDQAGTFWYHSHLSTQYCDGLRGPFVVYDPNDTHASLYDVDNDDTVITLADWYHTAAKLGPTFPLGADATLINGLGRSPSTTAADLAVINVTKGKRYRFRLVSLSCDPNHTFSIDGHDLTIIEVDSINSQPLVVDSIQIFAAQRYSFVLNADQDVGNYWIRANPSFGNVGFAGGINSAILRYDGADPVEPTTTQTTPTKPLNEVDLHPLDTMAVPGSPVAGGVDKAINMAFNFNGTNFFINGASFVPPTVPVLLQIISGAQNAQDLLPSGSVYSLPANADIEISFPATAAAPGAPHPFHLHGHAFAVVRSAGSTVYNYDNPIFRDVVSTGTPAAGDNVTIRFRTDNPGPWFLHCHIDFHLEAGFAVVMAEDIPDVASANPVPQAWSDLCPIYDALDVNDQ

SEQ ID NO: 23 - DNA, 1560 bp, Trametes sp.
atgtcgaggttccagtctcttctcgccttcgtcgtcgcctccctcgcggctgttgctcatgccgccattgggcccaccgctgacctcaccatctccaatgccgaggtcagccccgatgggttcgctcgtcaggccgtggttgtcaacaacgttaccccgggacccctggtcgcgggtaacaagggtgaccgcttccaactcaatgtcatcgacaacctcaccaaccacaccatgctgaagagcacgagtattcactggcacggctttttccagaaggggacgaactgggctgatggtcctgcgttcgtgaaccagtgccctatctcgtctgggcattcgttcctgtacgacttccaggttccggatcaggccggcacattctggtaccacagtcacttgtccacgcagtattgcgacggcctgcgcggtcccttcgttgtgtacgatccgaatgacccgcacgcgagcttgtatgacgtcgacaacgacgacaccgtgatcacgctcgcggattggtaccacaccgccgcaaagctcggaccagcattcccactgggtgccgacgcaacgctgatcaacgggcttggccgctccccaagcaccacggctgcggacctcgcagtcatcaacgtcacgaaggggaaacgctaccgtttccgcctcgtctccctgtcgtgtgatcccaaccacacgttcagtatcgatggtcatgacttgacgatcatcgaagtggactccatcaactcccagcatctggtggttgactccatccagatcttcgctgcgcagcggtactccttcgtgttgaatgccgaccaggatgtcggcaactactggattcgtgccaaccctagcttcggaaacgtcggatttgcgggcggtatcaactcggccatcctgcgctacgacggcgccgacccggtcgagcccaccacgacgcagactacgcccactaagcccctcaacgaggttgacctgcacccgctcgacaccatggctcccggctccccggtcgccggtggtgttgacaaggctatcaacatggccttcaacttcaacggtaccaacttcttcatcaacggcgcaagcttcgtgccccctaccgtgccggtcctgcttcagatcatcagcggtgctcaaaatgcccaggatcttcttccatctggcagtgtctactcgctcccggcgaacgctgacatcgagatctcgttccctgctaccgcggctgctccgggtgcccctcaccccttccacttgcacggtcacgcctttgccgtcgttcgcagcgctggcagcaccgtgtacaactacgacaaccccatcttccgcgacgtcgtcagcacggggacgcctgcggccggtgacaacgtgaccatccgcttccgcaccgacaaccctggcccgtggttcctccactgccacatcgacttccacttggaggccggttttgccgtcgtgatggcggaggacattcctgacgtcgcgtcggcgaacccggttccccaggcgtggtccgacctttgccccatctacgacgcgctcgatgtcaacgaccagtag

SEQ ID NO: 24 - protein, 519 aa, Trametes sp.
MSRFQSLLAFVVASLAAVAHAAIGPTADLTISNAEVSPDGFARQAVVVNNVTPGPLVAGNKGDRFQLNVIDNLTNHTMLKSTSIHWHGFFQKGTNWADGPAFVNQCPISSGHSFLYDFQVPDQAGTFWYHSHLSTQYCDGLRGPFVVYDPNDPHASLYDVDNDDTVITLADWYHTAAKLGPAFPLGADATLINGLGRSPSTTAADLAVINVTKGKRYRFRLVSLSCDPNHTFSIDGHDLTIIEVDSINSQHLVVDSIQIFAAQRYSFVLNADQDVGNYWIRANPSFGNVGFAGGINSAILRYDGADPVEPTTTQTTPTKPLNEVDLHPLDTMAPGSPVAGGVDKAINMAFNFNGTNFFINGASFVPPTVPVLLQIISGAQNAQDLLPSGSVYSLPANADIEISFPATAAAPGAPHPFHLHGHAFAVVRSAGSTVYNYDNPIFRDVVSTGTPAAGDNVTIRFRTDNPGPWFLHCHIDFHLEAGFAVVMAEDIPDVASANPVPQAWSDLCPIYDALDVNDQ

SEQ ID NO: 25 - DNA, 1563 bp, Lenzites gibbosa
atgtcgaggttccagactcttctcgctttcgtcgttacctccctcacagccgcggcgtatgctgccatcggacctgtggccgacctcaccatcactaatgccgaggtcagtcccgacgggttcgcccgtcaggctgtcgttgtcaacggcggtactcctggaccgcttgtgacggggaatatgggcgatcgcttccagcttaatgtgatcgacaacttgacaaaccacacgatgctgaaaagtaccagtattcactggcatgggttcttccaacacggcactaactgggccgatggtcctgctttcgtcaaccagtgcccaattgcatcggggcattcgttcttgtacgacttccaggtccccgaccaagccggtactttctggtaccacagtcacttgtccacgcagtactgcgatgggctgagaggccccttcgttgtctacgacccaaatgaccctcatgcaagcctctacgacgttgacaacgacgacactgtgataacactggcggattggtaccatgtcgcggcgaagctcggtcctcgtttcccgctgggcgcggatgcgactctgattaacgggctcggccgctctccaagtaccgtctctgcagacctctctgtgatcaatgtcacacctggtaaacgctaccggttccgccttgtatcgctgtcgtgcgacccgaaccacaccttcagcattgatggccacgatctgacgatcattgagaccgactccgtcaacactcaacctcttgtggtggattcaatccagatcttcgctgctcagcgatactccttcgtgttggaagccaaccagcccgtcgacaactattgggtccgtgcgaacccctccttcggaaacgtcgggttcagcggtggcatcaactctgccattttgcgatacgatggcgcccctgcagtagagcccacgacgacacagacaaccccaacgaagcctctcaacgaggttgacttgcacccgctcacgcctatgcctgtgcctggcgagcccgttgcgggaggtgttgacaagccgctcaacatggctttcaacttcaacggcaccagcttcttcatcaacggcgccagcttcgagcctcctaccgttccagttcttctccagattctcagtggcgcgcagacggctcaggagctactcccctccggaagcgtatacgtcctccccagcaatgcgtcgattgagatatccttcccggccactgcggccgcccctggagcacctcaccccttccacttgcacggtcacaccttcgctgttgtgcgcagcgccggcagtactgagtacaactacgacaaccccatcttccgcgacgtggtcagcacgggcacgcctgcggccggcgacaacgtcaccatccgtttccagacgaacaaccccgggccgtggttcctccactgccacatcgacttccacctcgacgccggcttcgcggtcgtcatggcggaggacatccctgatgtccaggcggtcaaccctgttccgcaggcgtggtccgacttgtgcccgatctacgatgcgctcgaccccagcgaccagtag

SEQ ID NO: 26 - protein, 520 aa, Lenzites gibbosa
MSRFQTLLAFVVTSLTAAAYAAIGPVADLTITNAEVSPDGFARQAVVVNGGTPGPLVTGNMGDRFQLNVIDNLTNHTMLKSTSIHWHGFFQHGTNWADGPAFVNQCPIASGHSFLYDFQVPDQAGTFWYHSHLSTQYCDGLRGPFVVYDPNDPHASLYDVDNDDTVITLADWYHVAAKLGPRFPLGADATLINGLGRSPSTVSADLSVINVTPGKRYRFRLVSLSCDPNHTFSIDGHDLTIIETDSVNTQPLVVDSIQIFAAQRYSFVLEANQPVDNYWVRANPSFGNVGFSGGINSAILRYDGAPAVEPTTTQTTPTKPLNEVDLHPLTPMPVPGEPVAGGVDKPLNMAFNFNGTSFFINGASFEPPTVPVLLQILSGAQTAQELLPSGSVYVLPSNASIEISFPATAAAPGAPHPFHLHGHTFAVVRSAGSTEYNYDNPIFRDVVSTGTPAAGDNVTIRFQTNNPGPWFLHCHIDFHLDAGFAVVMAEDIPDVQAVNPVPQAWSDLCPIYDALDPSDQ

SEQ ID NO: 27 - DNA, 1563 bp, Trametes hirsuta
atgtcgaggtttcagtctcttctgaccttcatcaatatttcccttgttgcggttgctcatgcagcggttggccctgttgccgacctcaccatcaccgacgcggcggtcagccctgacggtttctctcgccaggctgttgtggtgaacggcgtcacccctggaccgctcgttgcgggcaatattggggaccgcttccagctcaacgtcattgacaacttgacgaaccataccatgctcaagtcgaccagtattcactggcacggctttttccagcatggcacgaactgggctgatggtccggcgttcattaaccagtgccctatctctcctgggcactcgttcttgtacgacttccaggtacctgaccaagccggtaccttctggtaccacagtcacttgtcgacccagtactgtgatggtttgaggggccccttcgttgtctacgacccgaacgatccccatgccagccgctacgacgtcgacaacgacgacacggtcattactctggccgactggtaccataccgctgccaagctcgggccccggttcccggggggcgcggacgctactctcattaatggcaagggccgcgctcccagtgactctcccgccgagctgtcggtgatcaaggtcacgaagggcaaacgctaccgtttccgcttggtctcgctgtcatgcaaccccaaccataccttcagcattgatggtcacaacttgactatcatcgaggtcgacagtgtcaactcccagccgctggaagttgactccattcagatctttgcggcgcagcgctactccttcgtactggacgccaaccaggccgtcgacaactactggatccgggccaacccaaacttcggaaatgtcggattcgatgggggtattaactcggctatcctgcgctatgacggcgcgcccgctgttgagcccaccacgaaccagactacctcggttaagccgctgaacgaggtcgacctgcaccctcttgtctctaccccagtgcccgggagtccttcgtccggaggcgtcgacaaggcgatcaacatggctttcaacttcaacggctccaacttcttcatcaacggcgccagcttcgtcccgcccaccgtgcctgtcctgctccagattctcagtggtgcccagacggcgcaggacctcctgccctccggcagtgtatacgtccttccgtcgaacgcgtccattgagatctcgttccccgctacggccgccgcccctggtgctccccaccccttccacttgcacggtcacactttcgctgttgtgcgcagcgccggcagcaccgtgtacaactacgacaaccccatcttccgtgacgtcgtgagcacgggtacccctgcagcgggtgacaacgtcaccatccgcttcgacaccaacaacccaggcccgtggttccttcactgccacatcgacttccacttggagggtggctttgcggtcgtcatggctgaggatactccggacgtcaaggctgtcaaccccgtccctcaggcgtggtccgatctgtgcccgacctacgacgcgctcgaccccaacgaccagtaa

SEQ ID NO: 28 - protein, 520 aa, Trametes hirsuta
MSRFQSLLTFINISLVAVAHAAVGPVADLTITDAAVSPDGFSRQAVVVNGVTPGPLVAGNIGDRFQLNVIDNLTNHTMLKSTSIHWHGFFQHGTNWADGPAFINQCPISPGHSFLYDFQVPDQAGTFWYHSHLSTQYCDGLRGPFVVYDPNDPHASRYDVDNDDTVITLADWYHTAAKLGPRFPGGADATLINGKGRAPSDSPAELSVIKVTKGKRYRFRLVSLSCNPNHTFSIDGHNLTIIEVDSVNSQPLEVDSIQIFAAQRYSFVLDANQAVDNYWIRANPNFGNVGFDGGINSAILRYDGAPAVEPTTNQTTSVKPLNEVDLHPLVSTPVPGSPSSGGVDKAINMAFNFNGSNFFINGASFVPPTVPVLLQILSGAQTAQDLLPSGSVYVLPSNASIEISFPATAAAPGAPHPFHLHGHTFAVVRSAGSTVYNYDNPIFRDVVSTGTPAAGDNVTIRFDTNNPGPWFLHCHIDFHLEGGFAVVMAEDTPDVKAVNPVPQAWSDLCPTYDALDPNDQ

SEQ ID NO: 29 - DNA, 1563 bp, Lenzites gibbosa
atgtcgaggttccagactcttctcgckttcgtcgttacctccctcacagccgcggcgtatgctgccatcggacctgtggccgacctcaccatcactaatgccgaggtcagtcccgacgggttcgcccgtcaggctgtcgttgtcaacggcggtactcctggaccgcttgtgacggggaatatgggcgatcgcttccagcttaatgtgatcgacaacttgacaaaccacacgatgccgaaaagtaccagtattcactggcatgggttcttccaacacggcactaactgggccgatggtcctgctttcgtcaaccagtgcccaattgcatcggggcattcgttcttgtacgacttccaggtccccgaccaagccggtactttctggtaccacagtcacttgtccacgcagtactgcgatgggctgagaggccccttcgttgtctacgacccaaatgaccctcatgcaagcctctacgacgttgacaacgacgacactgtgataacactggcggattggtaccatgtcgcggcgaagctcggtcctcgtttcccgctgggcgcggatgcgactctgattaacgggctcggccgctctccaagtaccgtctctgcagacctctctgtgatcaatgtcacacctggtaaacgctaccggttccgccttgtatcgctgtcgtgcgacccgaaccataccttcagcatcgatgggcataacatgactatcatcgaagtcgatggtatcaacagcaagcccctcacggttgactccatccagatcttcgcagcgcaacgctactcattcgtgctgaacgcccatcaaactgtgaataactactggatccgtgctaaccccagctttggcacgaccgggttcgccggaggtatcaactctgccatcctgcgctacgacggtgcgcccgccgtcgagccgaccacgacgcagactgcctccgtcatcccactggtggagacgaacttgcacccgcttgtgcacatgcctgtgcctggtctgccaacgcccggcggtgttgacaagccgctcaacttcgcgttcaactttaacggcaccaactccttcatcaacaatgcatcattcacgccgccaacagtccctgtgttgctgcagatcctgagtggggcacatacggctcaggaactcctgccgcccgggtccgtgtacacgctcccgggccactcctctatcgagatcaccatgcccgcgacctccttggccccaggcgctccgcacccgttccacctgcacggccacgcgttcgcggtcgtgcgcagcgccggcagcaccgagtacaactacgacgatccgatcttccgcgacgtcgtcagcacaggcacgcccgccgcgggcgacaacgtcaccatccgcttccggacggacaaccccgggccgtggttcctccactgccacatcgacttccacctcaacgccggcttcgcggtcgtcatggcggaggacatccctgatgtccaggcggtcaaccctgttccgcaggcgtggtccgacttgtgcccgatctacgatgcgctcgaccccagcgaccagtag

SEQ ID NO: 30 - protein, 520 aa, Lenzites gibbosa
MSRFQTLLAFVVTSLTAAAYAAIGPVADLTITNAEVSPDGFARQAVVVNGGTPGPLVTGNMGDRFQLNVIDNLTNHTMPKSTSIHWHGFFQHGTNWADGPAFVNQCPIASGHSFLYDFQVPDQAGTFWYHSHLSTQYCDGLRGPFVVYDPNDPHASLYDVDNDDTVITLADWYHVAAKLGPRFPLGADATLINGLGRSPSTVSADLSVINVTPGKRYRFRLVSLSCDPNHTFSIDGHNMTIIEVDGINSKPLTVDSIQIFAAQRYSFVLNAHQTVNNYWIRANPSFGTTGFAGGINSAILRYDGAPAVEPTTTQTASVIPLVETNLHPLVHMPVPGLPTPGGVDKPLNFAFNFNGTNSFINNASFTPPTVPVLLQILSGAHTAQELLPPGSVYTLPGHSSIEITMPATSLAPGAPHPFHLHGHAFAVVRSAGSTEYNYDDPIFRDVVSTGTPAAGDNVTIRFRTDNPGPWFLHCHIDFHLNAGFAVVMAEDIPDVQAVNPVPQAWSDLCPIYDALDPSDQ

SEQ ID NO: 31 - DNA, 1563 bp, Trametes versicolor
atgtcgaggtttcactctcttctcgctttcgtcgttgcttcccttgcggctgtggcccacgctggtatcggtcctgtcgccgacctcaccatcaccaacgcagcagtcagccccgacgggttttctcgccaggccgtcgtcgtgaacggcggcacccctggccctctcatcaccggtaacatgggggatcgcttccagctcaatgtcatcgacaacctcacgaaccacacgatgctgaagagcaccagtattcactggcacggtttcttccagaagggcaccaactgggccgacggtcccgccttcatcaaccagtgcccgatctcatctggccactcgttcctgcatgacttccaggctcctgaccaggctggcaccttctggtatcacagtcacttgtccacgcagtactgtgatggtctgaggggtccgttcgttgtttacgaaccgaacgacccggccgccgacctgtacgacgtcgacaacgacgacacggtcattacccttgcggattggtaccacgtcgccgcgaagctgggccccgcactccctctcggcgccgacgcatctcacaacatcggtaagggacgctcccccagcacgaccaccgcggatcctatctgtattacgtgtatccccgggcaaacgtatccgtttccgcctggtgtccctgtcgtgcgaccccaaccacaccttcagcatcgatggtcacaacaagacgatcatcgattccgactcaatcaacacggcgcctcccgtggttcgaactcaattcgttctgtcgcccagcgtttctccttcgtgctcgaggccaaccaggccgtcgacaactactggattcgcgccaacccaaacttcggtaacgtcgggtttaccggcggcatcaactcggctatcctccgctttgatggcgccgctgccatggagcccaccaccacgcagaccacttcgaccgagccgctcaacggggtcaacctgcacccgctggttgccaccgctgtccctggctctcccgctgcgggtggtgttgacctggccatcaatatggcgttcaacttcaatggcaccaacttcttcatcaacggcgcgtctttcacgcccccgaccgtgcctgtcctcctccagatcatcagcggcgcgcagaacgcgcaggacctcctgcactccggcagcgtctactcgctccccccgaacgccgacattgagatctccttccccgccaccgctgccgcccccggtgcgctccaccccttccacttgcacgggcacgcgttcgcggtcgtccgcagcgccggcagcacggtctacaactacgacaaccccatcttccgcgacgtcgtcagcacggggaaccgtgcggccggtgacaacgtcaccatccgcttccgcaccgacaaccccggcccgtggttcctccactgccacatcgacttccacctcgaggccggctttgccgtcgtgttcgcggaagacatccccgacgtcgcgtcggcgaaccccgtcccccaggcgtggtccgacctgtgcccgacctacgacgcgcgcgacccgagcgaccagtaa

SEQ ID NO: 32 - protein, 520 aa, Trametes versicolor
MSRFHSLLAFVVASLAAVAHAGIGPVADLTITNAAVSPDGFSRQAVVVNGGTPGPLITGNMGDRFQLNVIDNLTNHTMLKSTSIHWHGFFQKGTNWADGPAFINQCPISSGHSFLHDFQAPDQAGTFWYHSHLSTQYCDGLRGPFVVYEPNDPAADLYDVDNDDTVITLADWYHVAAKLGPALPLGADASHNIGKGRSPSTTTADPICITCIPGQTYPFPPGVPVVRPQPHLQHRWSQQDDHRFRLNQHGASRGSNSIRSVAQRFSFVLEANQAVDNYWIRANPNFGNVGFTGGINSAILRFDGAAAMEPTTTQTTSTEPLNGVNLHPLVATAVPGSPAAGGVDLAINMAFNFNGTNFFINGASFTPPTVPVLLQIISGAQNAQDLLHSGSVYSLPPNADIEISFPATAAAPGALHPFHLHGHAFAVVRSAGSTVYNYDNPIFRDVVSTGNRAAGDNVTIRFRTDNPGPWFLHCHIDFHLEAGFAVVFAEDIPDVASANPVPQAWSDLCPTYDARDPSDQ

SEQ ID NO: 33 - DNA, 1563 bp, Trametes sp.
atgtcgaggttccactcccttcttacttttatcgtcgcctctttggcctcctcggcccttgcttccattgggcctgtcgccgacatgaccatttccaacgcggaagtgagccctgacgggtttgctcgtcaggctgtcgttgtcaacggtgtcacccccggacccctggtaaaggggaacatgggcgaccggttccagcttaatgttatcgacaatttgaccaaccacaccatgttgaagagtaccagtattcactggcacggtcttttccagcacggcaccaactgggcggacggaccggctttcgtgaaccagtgccctgtctccgcgggacactcgttcctgtacgatttccaggttccgggccaagcgggaactttctggtaccacagccatctgtccactcaatactgtgatggtttgaggggccctctcgttgtctacgaccctcatgaccctcacaagagtcgttacgacgtcgacaacgatgacacggttatcacgttggcggactggtaccacgtagcggcgaagcgtcggtccgcgtttcccctgggtgcggacgctactctcatcaacggtctcggtcgctccccgaccacccccagcgctgacctcgccgttatcaacgttacccagggcaagcggtaccgcttccgtctggtgtcgctgtcttgcgaccccaaccacacgttcagcattgacggtcacaacatgaccatcatcgaggttgattcggtcaactctcagcccctggtggtggattcgatccaaatcttcgctgcccagcgttactcgtttgtgcttaacgccaaccaagcggtcgacaactactgggtccgcgccaacccctcgttcggtaacgtcgggttctctggtggtatcaactcggctatcctgcggtacgctggtgcccctgctattgagcctaccacgaaccaaactacgtcggtcatccctctgaatgaggtcaacctgcaccctctggcccccacgcccgtgcccggaaaggccgtcgcgggtggtgttgacacaccgatcaacatggctttcagctttaacggcaccaacttcttcatcaacggcgcgagcttcgtaccccccactgtccctgtccttcttcagatcttgagtggcgcgcagtcggcccaggacctcctcccgtctggcagcgtctacgttctccccagcaacgcgtccattgaaatttccttccccgctaccgccgccgctcccggtgttccccaccccttccacttgcacggtcacacctttgctgtcgtccgcagcgctggcagcactgagtacaactacgacaaccccatcttccgcgacgtggtcagcacgggcacgcctgcggccggtgacaacgtcaccatccgcttccagaccaacaaccctggcccgtggttcctccactgccacatcgacttccatctcgaggccggtttcgcagtcgtcatggctgaggacactcccgacgtcaaggcggtcaaccccgttccccagtcgtggtccgacctctgccccatctacgatgcgcttgacgccagcgaccagtaa

SEQ ID NO: 34 - protein, 520 aa, Trametes sp.
MSRFHSLLTFIVASLASSALASIGPVADMTISNAEVSPDGFARQAVVVNGVTPGPLVKGNMGDRFQLNVIDNLTNHTMLKSTSIHWHGLFQHGTNWADGPAFVNQCPVSAGHSFLYDFQVPGQAGTFWYHSHLSTQYCDGLRGPLVVYDPHDPHKSRYDVDNDDTVITLADWYHVAAKRRSAFPLGADATLINGLGRSPTTPSADLAVINVTQGKRYRFRLVSLSCDPNHTFSIDGHNMTIIEVDSVNSQPLVVDSIQIFAAQRYSFVLNANQAVDNYWVRANPSFGNVGFSGGINSAILRYAGAPAIEPTTNQTTSVIPLNEVNLHPLAPTPVPGKAVAGGVDTPINMAFSFNGTNFFINGASFVPPTVPVLLQILSGAQSAQDLLPSGSVYVLPSNASIEISFPATAAAPGVPHPFHLHGHTFAVVRSAGSTEYNYDNPIFRDVVSTGTPAAGDNVTIRFQTNNPGPWFLHCHIDFHLEAGFAVVMAEDTPDVKAVNPVPQSWSDLCPIYDALDASDQ

SEQ ID NO: 35 - DNA, 1557 bp, Trametes sanguinea
atgtcgaggttccagtctctcctctccttcgtcctcgtctcccttgccgccgtggcgaacgctgccatcggccctgtggcagacctgaccctcaccaatgccgcggtcagccctgatggcttcagccgtgaggctgtcgtggtcaacggccaaacccctgggcctctcattgccggtcagaaaggcgaccgtttccagctgaatgtcattgacaatctgacgaaccacaccatgttgaagaccaccagtatccactggcatggcttcttccagcatggaacaaactgggccgacggccctgcgttcattaaccagtgtcccattgcatccggtcattccttcttatacgactttcaggttcctgaccaagcaggaaccttctggtaccacagccatctttccacgcagtactgcgatggtttgagggggccattcgttgtctatgatcccaacgatccccaggctagcctctatgacatagataatgatgacacggtcatcactttggccgattggtaccacgtcgccgctaaactcgggccacgcttcccgcttggggccgacgcgaccctcattaatggactcggtcgtagccccggtacgactgcggctgacttggctgtgatcaaagtcacacagggcaagcggtaccgtttccgcttggtgtctctctcttgcgacccgaatcataccttcagcattgatggccacactatgaccatcatcgagacagactcagtgaacactcagcctctggaggtcgactcgatccagatcttcgccgcacagcggtactcattcgtgctggatgccaaccagccggtagacaactactggatacgtgccaacccttccttcgggaacaccgggttcgccggcgggattaactccgccatcctccggtatgacggcgcgcccgaggtcgagcctaccacgaaccagaccactcctacgaagcctctgaacgaggttgacttgcacccgctcacccctatggctgtgcctggccttcccgagcccggaggtgttgacaagcctctgaacatggtcttcaactttaacggcacgaacttcttcatcaacggcgaatccttcgtcccaccctctgttccggtcttgctccagattctgagcggtgctcaggcagcacaagatctggttccgtcaggcagcgtttatgtgcttcccagcaactcgaccatcgaaatttccttccctgcgactgccaatgctcctggcgcaccgcacccgttccacctgcacggtcataccttcgctgtcgtccgaagcgcaggaagcagcgagtacaactacgataacccgatcttccgcgacgttgtcagcaccggtacgcccggcgataatgtcaccatccgcttcgagaccaacaaccccggcccgtggttcctccattgccacattgacttccacctggatgccggctttgctgtcgtcatggccgaggacactccggacacggcggcggccaaccctgtcccccagtcgtggtcggatttgtgcccgatctacgacgcgcttgaccctagcgatctctga

SEQ ID NO: 36 - protein, 518 aa, Trametes sanguinea
MSRFQSLLSFVLVSLAAVANAAIGPVADLTLTNAAVSPDGFSREAVVVNGQTPGPLIAGQKGDRFQLNVIDNLTNHTMLKTTSIHWHGFFQHGTNWADGPAFINQCPIASGHSFLYDFQVPDQAGTFWYHSHLSTQYCDGLRGPFVVYDPNDPQASLYDIDNDDTVITLADWYHVAAKLGPRFPLGADATLINGLGRSPGTTAADLAVIKVTQGKRYRFRLVSLSCDPNHTFSIDGHTMTIIETDSVNTQPLEVDSIQIFAAQRYSFVLDANQPVDNYWIRANPSFGNTGFAGGINSAILRYDGAPEVEPTTNQTTPTKPLNEVDLHPLTPMAVPGLPEPGGVDKPLNMVFNFNGTNFFINGESFVPPSVPVLLQILSGAQAAQDLVPSGSVYVLPSNSTIEISFPATANAPGAPHPFHLHGHTFAVVRSAGSSEYNYDNPIFRDVVSTGTPGDNVTIRFETNNPGPWFLHCHIDFHLDAGFAVVMAEDTPDTAAANPVPQSWSDLCPIYDALDPSDL

SEQ ID NO: 37 - DNA, 1557 bp, Pycnoporus coccineus
atgtcgaggttccagtctcttctctccttcgtcctcgtctcccttgccgccgtggcgaacgctgccatcggccctgtggcagacttgaccctcaccaatgccgcggtcagccctgatggcttcagccgtgaggctgtcgtggtcaacggccaaacccctgggcctctcattgccggtcagaaaggcgaccgtttccagctgaatgtcattgacaatttgacgaaccacaccatgttgaagaccaccagtatccactggcatggcttcttccagcatggcacaaactgggccgacggccccgcgttcatcaaccagtgtcccattgcatccggtcattccttcttatacgactttcaggttcctgaccaagcagggaccttctggtaccacagccatctttccacgcagtactgcgatggtttgagggggccgttcgttgtctatgatcccaacgatccccaggctagcctctatgacatagataatgatgacacggtcattactttggttgattggtaccacgtcgccgctaaactggggccacgcttcccgcttggggccgacgcgaccctcatcaatggactcggtcgtagccccggtacgactgcggctgacttggctgtgatcaaagtcacacagggcaagcggtaccgtttccgcttggtgtctctctcttgcgacccgaatcataccttcagcattgatggccacaccatgaccatcatcgaggcagactcagtgaacacacaacctcttgaggttgactcgatccagatcttcgccgcgcagcggtactccttcgtgctggatgccagccagcccgtggacaactactggatccgcgccaatccttccttcggaaacaccgggttcgccggtgggattaactccgccatcctccggtatgacggcgcgcccgaggtcgagcctaccacgacccagaccacttccacgaagcctctgaacgaggttgacttgcacccgctcacccctatggctgtgcctggccgtcccgagcccggaggtgttgacacaccgctgaacatggtcttcaactttaacggcacgaatttcttcatcaacgaccactccttcgtcccaccttctgttccggtcttgctccagattctgagcggtgcccaggcagcacaagatctggccccgtcaggtagcgtctatgtgcttcccagcaactcgtccatcgaaatctccttccctgcgactgccaatgctcctggcgcgccgcacccgttccacctgcacggtcataccttcgctgtcgtccgaagcgcaggaagcagcgagtacaactacgataacccgatcttccgcgacgttgtcagcaccggtacgcccggcgataatgtcaccatccgcttccagaccaacaaccctggcccgtggttcctccattgccacattgacttccacttggatgccggctttgctgtcgtcatggccgaggacactccggacacggcggcggccaaccctgtcccccagtcgtggtcggatttgtgcccgatctacgacgcgcttgaccctagcgatctctga

SEQ ID NO: 38 - protein, 518 aa, Pycnoporus coccineus
MSRFQSLLSFVLVSLAAVANAAIGPVADLTLTNAAVSPDGFSREAVVVNGQTPGPLIAGQKGDRFQLNVIDNLTNHTMLKTTSIHWHGFFQHGTNWADGPAFINQCPIASGHSFLYDFQVPDQAGTFWYHSHLSTQYCDGLRGPFVVYDPNDPQASLYDIDNDDTVITLVDWYHVAAKLGPRFPLGADATLINGLGRSPGTTAADLAVIKVTQGKRYRFRLVSLSCDPNHTFSIDGHTMTIIEADSVNTQPLEVDSIQIFAAQRYSFVLDASQPVDNYWIRANPSFGNTGFAGGINSAILRYDGAPEVEPTTTQTTSTKPLNEVDLHPLTPMAVPGRPEPGGVDTPLNMVFNFNGTNFFINDHSFVPPSVPVLLQILSGAQAAQDLAPSGSVYVLPSNSSIEISFPATANAPGAPHPFHLHGHTFAVVRSAGSSEYNYDNPIFRDVVSTGTPGDNVTIRFQTNNPGPWFLHCHIDFHLDAGFAVVMAEDTPDTAAANPVPQSWSDLCPIYDALDPSDL

SEQ ID NO: 39 - DNA, 1548 bp, Trametes hirsuta
atgtcgaggttccagtcgttgcttaccttcatcaccatctccctcgtcgcggttgctcatgcggcggttggccctgtcgccgacctcaccatcaccgacgcggcggtcagccctgacggtttctctcgccaggctgttgtggtgaacggcgtcacccctggaccgctcgttgcgggcaacattggggaccgcttccagctcaacgtcattgacaacttgacgaaccataccatgctcaagtcgaccagtatccactggcacggcttcttccagcatggcacgaactgggctgatggtccggcgttcattaaccagtgccctatctctcctgggcactcgttcttgtacgacttccaggtacctgaccaagccggtaccttctggtaccacagtcacttgtcgacccagtactgtgatggtttgaggggccccttcgttgtctacgacccgaacgatccccatgccagccgctacgacgtcgacaacgacgacacggtcattactctggccgactggtatcataccgctgccaagctaggtccccggttcccgggtgcggccgacgccgtcaacatcaacggcaagggccgcgccccagtgacactaccggcgagctgttcggtgatcaaggtcacgaagggcaaacgctaccgtttccgcttggtctcgctgtcatgcaaccccaaccataccttcagcattgatggtcacaacttgactatcatcgaggtcgacagtgtcaactcccagccgctggaggttgactccatccagatcttcgcggcgcaacgttactccttcgtgctggatgccaaccaggccgtcgacaactactggattcgggccaaccccaacttcggaaatgttggattcgacgggggtatcaactcggccatcctgcgctatgacggcgcgcccgctgtcgagcccaccacgaaccagactacctccgttaagccgctgaacgaggtcgacctgcaccctcttgtctctaccccggtgccaggcgcgagcgacaaggcgatcaacatggctttcaactttaatggctccaacttcttcatcaacggcgccagtttcgtcccgcccaccgtgcctgtcctcctccagattctcagtggtgcccagacggcgcaggacctcctgccctccggcagtgtatacgtccttccgtcgaacgcgtccattgagatctcgttccccgctaccgccgccgcccctggtgctccccatcccttccacttgcacggtcacactttcgctgttgtgcgcagcgccggcagcaccgtgtacaactacgacaatcccatcttccgtggcgtcgtgagcccaggtacccctgcagcgcgagacaacgtcaccatccgcttcgacaccaaccaacccggcccgtggttcctccactgccacatcgactttcacttggagggtggctttgcggtcgtcatggctgaggatactccggacgtacaggctgtcaaccccgttcctcaggcgtggtccgacctgtgcccgacctacgacgcgctcgaccccaacgaccagtaa

SEQ ID NO: 40 - protein, 515 aa, Trametes hirsuta
MSRFQSLLTFITISLVAVAHAAVGPVADLTITDAAVSPDGFSRQAVVVNGVTPGPLVAGNIGDRFQLNVIDNLTNHTMLKSTSIHWHGFFQHGTNWADGPAFINQCPISPGHSFLYDFQVPDQAGTFWYHSHLSTQYCDGLRGPFVVYDPNDPHASRYDVDNDDTVITLADWYHTAAKLGPRFPGAADAVNINGKGRAPVTLPASCSVIKVTKGKRYRFRLVSLSCNPNHTFSIDGHNLTIIEVDSVNSQPLEVDSIQIFAAQRYSFVLDANQAVDNYWIRANPNFGNVGFDGGINSAILRYDGAPAVEPTTNQTTSVKPLNEVDLHPLVSTPVPGASDKAINMAFNFNGSNFFINGASFVPPTVPVLLQILSGAQTAQDLLPSGSVYVLPSNASIEISFPATAAAPGAPHPFHLHGHTFAVVRSAGSTVYNYDNPIFRGVVSPGTPAARDNVTIRFDTNQPGPWFLHCHIDFHLEGGFAVVMAEDTPDVQAVNPVPQAWSDLCPTYDALDPNDQ

SEQ ID NO: 41 - DNA, 1563 bp, Trametes sp.
atgtcgaggttccactcccttcttacttttatcgtcgcctctttggcctcctcggcccttgcttccattgggcctgtcgccgacatgaccatttccaacgcggaagtgagccctgacgggtttgctcgtcaggctgtcgttgtcaacggtgtcacccccggacccctggtaaaggggaacatgggcgaccggttccagcttaatgttatcgacaatttgaccaaccacaccatgttgaagagtaccagtattcactggcacggtcttttccagcacggcaccaactgggcggacggaccggctttcgtgaaccagtgccctgtctccgcgggacactcgttcctgtacgatttccaggttccgggccaagcgggaactttctggtaccacagccatctgtccactcaatactgtgatggtttgaggggccctctcgttgtctacgaccctcatgaccctcacaagagtcgttacgacgtcgacaacgatgacacggttatcacgttggcggactggtaccacgtagcggcgaagcgtcggtccgcgtttccgctgggtgcggacgctactctcatcaacggtctcggtcgctccccgaccacccccagcgctgacctcgccgttatcaacgttacccagggcaagcggtaccgcttccgtctggtgtcgctgtcttgcgaccccaaccacacgttcagcattgacggtcacaacatgaccatcatcgaggttgattcggtcaactctcagcccctggtggtggattcgatccaaatcttcgctgcccagcgttactcgtttgtgcttaacgccaaccaagcggtcgacaactactgggtccgcgccaacccctcgttcggtaacgtcgggttctctggtggtatcaactcggctatcctgcggtacgctggtgcccctgctattgagcctaccacgaaccaaactacgtcggtcatccctctgaatgaggtcaacctgcaccctctggcccccacgcccgtgcccggaaaggccgtcgcgggtggtgttgacacaccgatcaacatggctttcagctttaacggcaccaacttcttcatcaacggcgcgagcttcgtaccccccactgtccctgtccttcttcagatcttgagtggcgcgcagtcggcccaggacctcctcccgtctggcagcgtctacgttctccccagcaacgcgtccattgaaatttccttccccgctaccgccgccgctcccggtgttccccaccccttccacttgcacggtcacacctttgctgtcgtccgcagcgctggcagcactgagtacaactacgacaaccccatcttccgcgacgtggtcagcacgggcacgcctgcggccggtgacaacgtcaccatccgcttccagaccaacaaccctggcccgtggttcctccactgccacatcgacttccatctcgaggccgggttcgcagttgtcatggctgaggacactcccgacgtcaaggcggtcaaccccgttccccagtcgtggtccgacctctgccccatctacgatgcgcttgacgccagcgacctctaa

SEQ ID NO: 42 - protein, 520 aa, Trametes sp.
MSRFHSLLTFIVASLASSALASIGPVADMTISNAEVSPDGFARQAVVVNGVTPGPLVKGNMGDRFQLNVIDNLTNHTMLKSTSIHWHGLFQHGTNWADGPAFVNQCPVSAGHSFLYDFQVPGQAGTFWYHSHLSTQYCDGLRGPLVVYDPHDPHKSRYDVDNDDTVITLADWYHVAAKRRSAFPLGADATLINGLGRSPTTPSADLAVINVTQGKRYRFRLVSLSCDPNHTFSIDGHNMTIIEVDSVNSQPLVVDSIQIFAAQRYSFVLNANQAVDNYWVRANPSFGNVGFSGGINSAILRYAGAPAIEPTTNQTTSVIPLNEVNLHPLAPTPVPGKAVAGGVDTPINMAFSFNGTNFFINGASFVPPTVPVLLQILSGAQSAQDLLPSGSVYVLPSNASIEISFPATAAAPGVPHPFHLHGHTFAVVRSAGSTEYNYDNPIFRDVVSTGTPAAGDNVTIRFQTNNPGPWFLHCHIDFHLEAGFAVVMAEDTPDVKAVNPVPQSWSDLCPIYDALDASDL

SEQ ID NO: 43 - DNA, 1557 bp, Pycnoporus coccineus
atgtcgaggttccagtctcttctctccttcgtcctcgtctcccttgccgccgtggcgaacgctgccatcggccctatggcagacttgaccctcaccaatgccgcggtcagccctgatggcttcagccgtgaggctgtcgtggtcaacggccaaacccctgggcctctcattgccggtcagaaaggcgaccgtttccagctgaatgtcattgacaatttgacgaaccacaccatgttgaagaccaccagtatccactggcatggcttcttccagcatggcacaaactgggccgacggccccgcgttcatcaaccagtgtcccattgcatccggtcattccttcttatacgactttcaggtccctgaccaagcagggaccttctggtaccacagccatctttccacgcagtactgcgatggtttgagggggccgttcgttgtctatgatcccaacgatccccaggctagcctctatgacatagataatgatgacacggtcattactttggttgattggtaccacgtcgccgctaaactggggccacgcttcccgcttggggcggacgcgaccctcatcaatggactcggtcgtagccccggtacgactgcggctgacttggctgtgatcaaagtcacacagggcaagcggtaccgtttccgcttggtgtctctctcttgcgacccgaatcataccttcagcattgatggccacaccatgaccatcatcgaggcagactcagtgaacacacaacctcttgaggttgactcgatccagatcttcgccgcgcagcggtactccttcgtgctggatgccagccagcccgtggacaactactggatccgcgccaatccttccttcggaaacaccgggttcgccggtgggattaactccgccatcctccggtatgacggcgcgcccgaggtcgagcctaccacgacccagaccacttccacgaagcctctgaacgaggttgacttgcacccgctcacccctatggctgtgcctggccgtcccgagcccggaggtgttgacacaccgctgaacatggtcttcaactttaacggcacgaatttcttcatcaacgaccactccttcgtcccaccttctgttccggtcttgctccagattctgagcggtgcccaggcagcacaagatctggccccgtcaggtagcgtctatgtgcttcccagcaactcgtccatcgaaatctccttccctgcgactgccaatgctcctggcgcgccgcacccgttccacctgcacggtcataccttcgctgtcgtccgaagcgcaggaagcagcgagtacaactacgataacccgatcttccgcgacgttgtcagcaccggtacgcccggcgataatgtcaccatccgcttccagaccaacaaccctggcccgtggttcctccattgccacattgacttccacttggatgccggctttgctgtcgtcatggccgaggacactccggacacggcagcggccaaccctgtcccccagtcgtggtcggatttgtgcccgatctacgacgcgcttgaccctagcgatctctga

SEQ ID NO: 44 - protein, 518 aa, Pycnoporus coccineus
MSRFQSLLSFVLVSLAAVANAAIGPMADLTLTNAAVSPDGFSREAVVVNGQTPGPLIAGQKGDRFQLNVIDNLTNHTMLKTTSIHWHGFFQHGTNWADGPAFINQCPIASGHSFLYDFQVPDQAGTFWYHSHLSTQYCDGLRGPFVVYDPNDPQASLYDIDNDDTVITLVDWYHVAAKLGPRFPLGADATLINGLGRSPGTTAADLAVIKVTQGKRYRFRLVSLSCDPNHTFSIDGHTMTIIEADSVNTQPLEVDSIQIFAAQRYSFVLDASQPVDNYWIRANPSFGNTGFAGGINSAILRYDGAPEVEPTTTQTTSTKPLNEVDLHPLTPMAVPGRPEPGGVDTPLNMVFNFNGTNFFINDHSFVPPSVPVLLQILSGAQAAQDLAPSGSVYVLPSNSSIEISFPATANAPGAPHPFHLHGHTFAVVRSAGSSEYNYDNPIFRDVVSTGTPGDNVTIRFQTNNPGPWFLHCHIDFHLDAGFAVVMAEDTPDTAAANPVPQSWSDLCPIYDALDPSDL

SEQ ID NO: 45 - DNA, 1557 bp, Cinnabarina coccineus
atgtcgagattccaatctctcctctcctttgtcctcgtctctcttgccgctgtggccaacgctgccatcggtcctgtggcagacttgaccctcaccaacgccgcggtcagccccgatggcttcagccgcgaggctgttgtggtcaatgggatcacccccgctcctctcattgctggacaaaaaggcgaccgtttccagctgaatgtcatcgacaatctgacgaaccataccatgctgaagactactagtatccactggcatggcttcttccagcacggtacgaattgggccgacggtgtgtcgttcgtcaaccagtgccccatcgcttcgggccattcgttcttgtacgacttccaggttcccgaccaagcagggacgttctggtatcacagccatctttccacccagtactgtgatggtttgcgggggcccttcgtcgtctacgaccccaatgatcctcaggctagcctgtatgacattgacaacgatgacactgtcattacattggccgactggtaccacgtcgccgctaagcttggcccacgcttcccgcttggcgcggatgcaactctcatcaacgggctgggtcgaagccccggtactaccactgctgatctggcagttatcaaggtcacgcagggcaagcggtaccgattccgtttggtgtccctttcttgcgacccgaaccacacctttagcatcgatggccacactatgactgtgatcgaggcggactcagtgaatactcagcccctcgaagttgactcgattcagatcttcgccgcccagcggtactccttcgtgctggatgctagccagcccgtcgacaactactggatccgtgctaaccctgctttcggaaacgtcggattcgccggtggaatcaactctgctattctgcggtatgacggcgcacccgaggtggagcctaccacgacccaaaccacttcgacgaagcctctcaacgaggctgacttgcatcccctcacccctatgcctgtgcctggtcgtcccgaggccggtggtgttgacaagcctctgaacatggtcttcaacttcaacggcaccaacttcttcatcaacaatcactcctttgtcccaccctccgtcccggttctgctccagattctcagcggtgctcaggccgcgcaggacctcgttccggacggcagcgtctacgttctcccgagcaactcgtctattgagatctccttccccgcaactgccaatgctcctggcacccctcaccccttccacctgcacggtcacaccttcgctgtcgtccgaagcgccggaagcagcgagtacaactacgataacccgatcttccgcgacgtcgtgagcaccggccagcccggagacaacgtcaccatccggttccagaccaacaaccccggcccctggttcctccactgccacatcgacttccacttggaagccggttttgctgtcgtcctggccgaggacactccagacacggcggcggtcaaccctgtcccccagtcgtggtcggatctgtgccccatctacgacgcacttgaccccagcgatctctga

SEQ ID NO: 46 - protein, 518 aa, Cinnabarina coccineus
MSRFQSLLSFVLVSLAAVANAAIGPVADLTLTNAAVSPDGFSREAVVVNGITPAPLIAGQKGDRFQLNVIDNLTNHTMLKTTSIHWHGFFQHGTNWADGVSFVNQCPIASGHSFLYDFQVPDQAGTFWYHSHLSTQYCDGLRGPFVVYDPNDPQASLYDIDNDDTVITLADWYHVAAKLGPRFPLGADATLINGLGRSPGTTTADLAVIKVTQGKRYRFRLVSLSCDPNHTFSIDGHTMTVIEADSVNTQPLEVDSIQIFAAQRYSFVLDASQPVDNYWIRANPAFGNVGFAGGINSAILRYDGAPEVEPTTTQTTSTKPLNEADLHPLTPMPVPGRPEAGGVDKPLNMVFNFNGTNFFINNHSFVPPSVPVLLQILSGAQAAQDLVPDGSVYVLPSNSSIEISFPATANAPGTPHPFHLHGHTFAVVRSAGSSEYNYDNPIFRDVVSTGQPGDNVTIRFQTNNPGPWFLHCHIDFHLEAGFAVVLAEDTPDTAAVNPVPQSWSDLCPIYDALDPSDL

SEQ ID NO: 47 - DNA, 1557 bp, Trametes cinnabarina
atgtccagattccaatctctcctctcctttgtcctcgtctctcttgccgctgtggccaacgctgccatcggtcctgtggcagacttgaccctcaccaacgccgcggtcagccccgatggcttcagccgcgaggctgttgtggtcaatgggatcacccccgctcctctcattgctggacaaaaaggcgaccgtttccagctgaatgtcatcgacaatctgacgaaccataccatgctgaagactactagtatccactggcatggcttcttccagcacggtacgaattgggccgacggtgtgtcgttcgtcaaccagtgccccatcgcttcgggccattcgttcttgtacgacttccaggttcccgaccaagcagggacgttctggtatcacagccatctttccacccagtactgtgatggtttgcgggggcccttcgtcgtctacgaccccaatgatcctcaggctagcctgtatgacattgacaacgatgacactgtcattacattggccgactggtaccacgtcgccgctaagcttggcccacgcttcccgcttggcgcggatgcaactctcatcaacgggctgggtcgaagccccggtactaccactgctgatctggcagtcatcaaggtcacgcagggcaagcggtaccgattccgtttggtgtccctttcttgcgacccgaaccacacctttagcatcgatggccacactatgactgtgatcgaggcggactcagtgaatactcagcccctcgaagttgactcgattcagatcttcgccgcccagcggtactccttcgtgctggatgctagccagcccgtcgacaactactggatccgtgctaaccctgctttcggaaacgtcggattcgccggtggaatcaactctgctattctgcggtatgacggcgcacccgaggtggagcctaccacgacccaaaccacttcgacgaagcctctcaacgaggctgacttgcatcccctcacccctatgcctgtgcctggtcgtcccgaggccggtggtgttgacaagcctctgagcatggtcttcaacttcaacggcaccaacttcttcatcaacaatcactcctttgtcccaccctccgtcccggttctgctccagattctcagcggtgctcaggccgcgcaggacctcgttccggacggcagcgtctacgttctcccgagcaactcgtctattgagatctccttccccgcaactgccaatgctcctggcacccctcaccccttccacctgcacggtcacaccttcgctgtcgtccgaagcgccggaagcagcgagtacaactacgataacccgatcttccgcgacgtcgtgagcaccggccagcccggagacaacgtcaccatccggttccagaccaacaaccccggcccctggttcctccactgccacatcgacttccacttggaagccggttttgctgtcgtcctggccgaggacactccagacacggcggcggtcaaccctgtcccccagtcgtggtcggatctgtgccccatctacgacgcacttgaccccagcgatctctga

SEQ ID NO: 48 - protein, 518 aa, Trametes cinnabarina
MSRFQSLLSFVLVSLAAVANAAIGPVADLTLTNAAVSPDGFSREAVVVNGITPAPLIAGQKGDRFQLNVIDNLTNHTMLKTTSIHWHGFFQHGTNWADGVSFVNQCPIASGHSFLYDFQVPDQAGTFWYHSHLSTQYCDGLRGPFVVYDPNDPQASLYDIDNDDTVITLADWYHVAAKLGPRFPLGADATLINGLGRSPGTTTADLAVIKVTQGKRYRFRLVSLSCDPNHTFSIDGHTMTVIEADSVNTQPLEVDSIQIFAAQRYSFVLDASQPVDNYWIRANPAFGNVGFAGGINSAILRYDGAPEVEPTTTQTTSTKPLNEADLHPLTPMPVPGRPEAGGVDKPLSMVFNFNGTNFFINNHSFVPPSVPVLLQILSGAQAAQDLVPDGSVYVLPSNSSIEISFPATANAPGTPHPFHLHGHTFAVVRSAGSSEYNYDNPIFRDVVSTGQPGDNVTIRFQTNNPGPWFLHCHIDFHLEAGFAVVLAEDTPDTAAVNPVPQSWSDLCPIYDALDPSDL

SEQ ID NO: 49 - DNA, 1557 bp, Trametes sanguinea
atgtcgaggttccagtccctcttcttcttcgtcctcgcttccctcgccgctgtggccaacgctgccatcggtcctgtggcagacttgaccctcaccaacgccgcagtcagccctgatggcttcacccgcgaggctgttgttgtcaacggcatcactcctgctcctctcattgccgggaagaaaggcgaccgcttccagctgaatgtcatcgacaatttgacaaaccataccatgctgaagaccaccagtattcactggcatggcttcttccaacacggcacgaactgggcagacggcgtgtcgttcgtcaaccagtgccccatcgcttcgggccattcgttcttgtacgacttccaggtccccgaccaagcaggaactttctggtatcacagtcatctttccacccagtattgtgatggattgagaggccccttcgtcgtctacgacccgaatgatccccaggccagcttgtatgacattgacaacgacgacactgtgattactttggccgactggtaccatcttgccgccaaagttggacagcgcttcccagttggcgcggatgcgactctgattaacgggcttggtcgaacccccggcacgacctctgctgatctggcggttatcaaggtcacacagggcaagcggtaccgattccgtttggtgtccctgtcttgcgacccgaaccataccttcagcatcgatggtcacaccatgaccgtcattgaagcggattcggtgaacacccagcccctcgaagttgactcaattcagatcttcgccgcacagcggtactccttcgtgctggatgctagtcagccggtggacaactactggatccgtgccaaccctcccttcggaaacgtcggattcgccggtggaatcaactctgctattctgcgatacgatggcgctcccgaggtcgagcccaccacgacccagaccactcccacgaagcctctgaatgaggctgacttgcatcctcttactcccatgcctgtgcctggacgccccgagcccggaggtgtcgacaagccgctcaacatggtcttcaacttcaacggcacgaacttcttcatcaacaaccattctttcgtcccaccctccgtgccggtcctgctccagattctcagcggcgctcaggccgcacaggacctggtcccggaaggcagcgtctacgttctcccgagcaacgcctctattgagatctccttccccgcaactgccaatgctcctggcagccctcaccccttccacctgcacggtcacaccttcgctgtcgtccgaagcgccggaagcagcgagtacaactacgacaacccggtcttccgcgacgtcgtgagcaccggtacgcccggcgacaacgtcaccatccggttccagaccaacaaccccggcccttggttcctccactgccacatcgacttccacttggatgccggctttgctgtcgtcatggccgaggacactccagacaccgcctcggtcaaccaggtccctcagtcatggtcggatttgtgcccgatctacgacgcgcttgacctcagcgacctctga

SEQ ID NO: 50 - protein, 518 aa, Trametes sanguinea
MSRFQSLFFFVLASLAAVANAAIGPVADLTLTNAAVSPDGFTREAVVVNGITPAPLIAGKKGDRFQLNVIDNLTNHTMLKTTSIHWHGFFQHGTNWADGVSFVNQCPIASGHSFLYDFQVPDQAGTFWYHSHLSTQYCDGLRGPFVVYDPNDPQASLYDIDNDDTVITLADWYHLAAKVGQRFPVGADATLINGLGRTPGTTSADLAVIKVTQGKRYRFRLVSLSCDPNHTFSIDGHTMTVIEADSVNTQPLEVDSIQIFAAQRYSFVLDASQPVDNYWIRANPPFGNVGFAGGINSAILRYDGAPEVEPTTTQTTPTKPLNEADLHPLTPMPVPGRPEPGGVDKPLNMVFNFNGTNFFINNHSFVPPSVPVLLQILSGAQAAQDLVPEGSVYVLPSNASIEISFPATANAPGSPHPFHLHGHTFAVVRSAGSSEYNYDNPVFRDVVSTGTPGDNVTIRFQTNNPGPWFLHCHIDFHLDAGFAVVMAEDTPDTASVNQVPQSWSDLCPIYDALDLSDL

SEQ ID NO: 51 - DNA, 1557 bp, Trametes cinnabarina
atgtcgaggttccagtccctcttcttcttcgtcctcgtctccctcaccgctgtggccaacgcagccatagggcctgtggcggacctgacccttaccaatgcccaggtcagccccgatggcttcgctcgcgaggccgtcgtggtgaacggtatcacccctgcccctctcatcacaggcaataagggcgatcgattccagctcaatgtcatcgaccagttgacaaatcataccatgttgaaaacatctagtattcattggcacggcttcttccagcaaggcacgaactgggccgatggtcccgcgttcgtgaaccagtgtcccatcgcttcgggccactcgttcttgtatgactttcaagttcccgaccaagcagggactttctggtaccatagccatctctccacgcaatactgcgatggtttgagggggcctttcgtcgtctacgaccccaacgatcctcacgctagcctgtatgacattgataacgacgacactgtcattacgctggctgattggtatcacgttgctgccaagctcggacctcgcttcccatttggctccgattcaacccttatcaatggacttggtcgaaccactggcatagcaccgtccgacttggcagttatcaaggtcacgcagggcaagcgctaccgcttccgcttggtgtcgctttcttgcgatccgaaccatacattcagcattgataatcacacaatgactataattgaggcggactcgatcaacactcaacccctagaggttgattcaatccagatttttgccgcgcagcgctactccttcgtgctggatgctagccagccggtggataactactggatccgcgcaaaccctgccttcggaaacacaggttttgctggtggaatcaattctgccatcctgcgttatgatggcgcacccgagatcgagcctacgtctgtccagactactcctacgaagcctctgaacgaggtcgacttgcatcctctctcgcctatgcctgtgcctggcagccccgagcccggaggtgtcgacaagcctctgaacttggtcttcaacttcaacggcaccaacttcttcatcaacgaccacacctttgtcccgccgtctgtcccagtcttgctacaaatcctcagtggggcgcaggcggctcaggacctggtcccggagggcagcgtgttcgttcttcccagcaactcgtccattgagatatccttccctgccactgccaatgcccctggattcccccatccgttccacttgcacggtcacgccttcgctgtcgtccggagcgccgggagcagcgtctacaactacgacaacccgatcttccgcgacgtcgtcagcaccggccagcccggcgacaacgtcacgattcgcttcgagaccaataacccaggcccgtggttcctccactgccacattgacttccacctcgacgcaggctttgctgtagtcatggccgaggacactccggacaccaaggccgcgaaccctgttcctcaggcgtggtcggacttgtgccccatctatgatgcacttgaccccagcgacctctga

SEQ ID NO: 52 - protein, 518 aa, Trametes cinnabarina
MSRFQSLFFFVLVSLTAVANAAIGPVADLTLTNAQVSPDGFAREAVVVNGITPAPLITGNKGDRFQLNVIDQLTNHTMLKTSSIHWHGFFQQGTNWADGPAFVNQCPIASGHSFLYDFQVPDQAGTFWYHSHLSTQYCDGLRGPFVVYDPNDPHASLYDIDNDDTVITLADWYHVAAKLGPRFPFGSDSTLINGLGRTTGIAPSDLAVIKVTQGKRYRFRLVSLSCDPNHTFSIDNHTMTIIEADSINTQPLEVDSIQIFAAQRYSFVLDASQPVDNYWIRANPAFGNTGFAGGINSAILRYDGAPEIEPTSVQTTPTKPLNEVDLHPLSPMPVPGSPEPGGVDKPLNLVFNFNGTNFFINDHTFVPPSVPVLLQILSGAQAAQDLVPEGSVFVLPSNSSIEISFPATANAPGFPHPFHLHGHAFAVVRSAGSSVYNYDNPIFRDVVSTGQPGDNVTIRFETNNPGPWFLHCHIDFHLDAGFAVVMAEDTPDTKAANPVPQAWSDLCPIYDALDPSDL

SEQ ID NO: 53 - DNA, 1575 bp, Trametes sp.
atgtcgggcttccgtctccttccttcattcgcgtcacttgctgtgatcgtgtcgctcgcgctcaacacgttcgcggcggtcggtcccgtgaccgacctgaccatctccaacgcgaacgtctcccccgacggtttccagcgtgcggcggtcgtcgcgaacggcggggtccctggcccgctcattaacggccagaagggtgaccatttccagatcaatgtggtcaaccagcttacgaaccacaccatgctcaagtccaccagtatccactggcacggtttcttccagaagggcacgaactgggcggacggtcctgccttcgtgaaccagtgtcctattgcaaccggccattcgttcctgtatgacttccaggtccccgatcaggctggtactttctggtatcacagccacttgtcgacgcagtactgtgatggtctgcgcggaccgttcgtcgtctacgacccgaatgatcctcatgccagcctttacgatgtggacaacgaggacaccgtcatcactctcgccgactggtatcatgttgcggcaaagcttgggccggcgttccctccccgcgccgatgccaccttgatcaatggcctcggtcgctcaacggatactccgaccgcggacttggccgtcatcaaggtcacgtcgggcaagcggtaccgtttccgtctggcatcgctttcttgcgaccccgcgttcactttcagcattgacaaccatgatatgactatcatcgaggccgatgctgtcaacactcagccgcttgaggtcgactcgctccagatctttgctggtcagcgttactcgttcgtcctcgaggcgaaccaggctgtcgacaactactgggttcgtgcgaacccattctttggtacgacgggctttgcgggcgggatcaactctgccatcctccgctacgatggcgccgccgaggtcgagccgactaccacgcaaagcacgtcgacgaagccgctcgctgaaaccgaccttgtgcccctggcgtcgatgccggttccgggttcccccgtgtctggtggagtcgacaaggcgatcaactttgcgttcaccttcaacggcaccaacttcttcgtgaacggcgcgaccttcacgcctcccagcactcctgttctgctgcagatcatgagcggtgcgcaggatgcctcggctcttctcccgtctggcgatgtctactccctgccctcgaacgccacgattgagctcaccttcccggccacgactggcgcacccggtgctcctcatcccttccacttgcacggtcacaccttcgccgttgttcgcagcgcaggcagcaccaagtacaactacgataacccgatctggcgcgatgttgttagcactggaactcctgccgcgggtgacaacgttactatccgcttcaggaccgacaaccccgggccatggttcctccactgccacatcgacttccacctcgaggccgggttcgccgttgtcatggccgaagacattcctgacactaagcttgccaaccctgttcctcaggcgtggtcggacctgtgcccgatctacgatgcgctcgaccccagcgaccagtga

SEQ ID NO: 54 - protein, 524 aa, Trametes sp.
MSGFRLLPSFASLAVIVSLALNTFAAVGPVTDLTISNANVSPDGFQRAAVVANGGVPGPLINGQKGDHFQINVVNQLTNHTMLKSTSIHWHGFFQKGTNWADGPAFVNQCPIATGHSFLYDFQVPDQAGTFWYHSHLSTQYCDGLRGPFVVYDPNDPHASLYDVDNEDTVITLADWYHVAAKLGPAFPPRADATLINGLGRSTDTPTADLAVIKVTSGKRYRFRLASLSCDPAFTFSIDNHDMTIIEADAVNTQPLEVDSLQIFAGQRYSFVLEANQAVDNYWVRANPFFGTTGFAGGINSAILRYDGAAEVEPTTTQSTSTKPLAETDLVPLASMPVPGSPVSGGVDKAINFAFTFNGTNFFVNGATFTPPSTPVLLQIMSGAQDASALLPSGDVYSLPSNATIELTFPATTGAPGAPHPFHLHGHTFAVVRSAGSTKYNYDNPIWRDVVSTGTPAAGDNVTIRFRTDNPGPWFLHCHIDFHLEAGFAVVMAEDIPDTKLANPVPQAWSDLCPIYDALDPSDQ

SEQ ID NO: 55 - DNA, 1575 bp, Trametes sp.
atgtcgggcttccgtctccttccttcattcgcgtcacttgctgtgatcgtgtcgctcgcgctcaacacgttcgcggcggtcggtcccgtgaccgacctgaccatctccaacgcgaacgtctcccccgacggtttccagcgtgcggcggtcgtcgcgaacggcggggtccctggcccgctcattaacggccagaagggtgaccatttccagatcaatgtggtcaaccagcttacgaaccacaccatgctcaagtccaccagtatccactggcacggtttcttccagaagggcacgaactgggcggacggtcctgccttcgtgaaccagtgtcctattgcaaccggccattcgttcctgtatgacttccaggtccccgatcaggctggtactttctggtatcacagccacttgtcgacgcagtactgtgatggtctgcgcggaccgttcgtcgtctacgacccgaatgatcctcatgccagcctttacgatgtggacaacgaggacaccgtcatcactctcgccgactggtatcatgttgcggcaaagcttgggccggcgttccctccccgcgccgatgccaccttgatcaatggcctcggtcgctcaacggatactccgaccgcggacttggccgtcatcaaggtcacgtcgggcaagcggtaccgtttccgtctggcatcgctttcttgcgaccccgcgttcactttcagcattgacaaccatgatatgactatcatcgaggccgatgctgtcaacactcagccgcttgaggtcgactcgctccagatctttgctggtcagcgttactcgttcgtcctcgaggcgaaccaggctgtcgacaactactgggttcgtgcgaacccattctttggtacgacgggctttgcgggcgggatcaactctgccatcctccgctacgatggcgccgccgaggtcgagccgactaccacgcaaagcacgtcgacgaagccgctcgctgaaaccgaccttgtgcccctggcgtcgatgccggttccgggttcccccgtgtctggtggagtcgacaaggggatcaactttgcgttcaccttcaacggcaccaacttcttcgtgaacggcgcgaccttcacgcctcccagcactcctgttctgctgcagatcatgagcggtgcgcaggatgcctcggctcttctcccgtctggcgatgtctactccctgccctcgaacgccacgattgagctcaccttcccggccacgactggcgcacccggtgctcctcatcccttccacttgcacggtcacaccttcgccgttgttcgcagcgcaggcagcaccaagtacaactacgataacccgatctggcgcgatgttgttagcactggaactcctgccgcgggtgacaacgttactatccgcttcaggaccgacaaccccggcccatggttcctccactgccacatcgacttccacctcgaggccggtttcgccgttgtcatggccgaggacattcctgacactaagcttgccaaccctgttcctcaggcgtggtcggacctgtgcccgatctacgatgcgctcgaccccagcgaccagtga

SEQ ID NO: 56 - protein, 524 aa, Trametes sp.
MSGFRLLPSFASLAVIVSLALNTFAAVGPVTDLTISNANVSPDGFQRAAVVANGGVPGPLINGQKGDHFQINVVNQLTNHTMLKSTSIHWHGFFQKGTNWADGPAFVNQCPIATGHSFLYDFQVPDQAGTFWYHSHLSTQYCDGLRGPFVVYDPNDPHASLYDVDNEDTVITLADWYHVAAKLGPAFPPRADATLINGLGRSTDTPTADLAVIKVTSGKRYRFRLASLSCDPAFTFSIDNHDMTIIEADAVNTQPLEVDSLQIFAGQRYSFVLEANQAVDNYWVRANPFFGTTGFAGGINSAILRYDGAAEVEPTTTQSTSTKPLAETDLVPLASMPVPGSPVSGGVDKGINFAFTFNGTNFFVNGATFTPPSTPVLLQIMSGAQDASALLPSGDVYSLPSNATIELTFPATTGAPGAPHPFHLHGHTFAVVRSAGSTKYNYDNPIWRDVVSTGTPAAGDNVTIRFRTDNPGPWFLHCHIDFHLEAGFAVVMAEDIPDTKLANPVPQAWSDLCPIYDALDPSDQ

SEQ ID NO: 57 - DNA, 1566 bp, Lentinus sp.
atggccaagttccagtcgttgctttcttacactgtcctctccttcgtcgcggctgcctatgctgccatcggcccagtcgctgaccttaccatcagcaatgcccaagtcagccccgacggcttcctccgcgatgccgtcgtgaccaacggcctggtccctgggcccctcatcacgggcaacaagggcgatcgcttccagttgaatgtcattgatcaaatgaccaaccacacgatgttgaagactacgagcattcactggcacggcttcttccagaagggcaccaactgggctgatggacctgcgtttgtgaaccagtgccccattgccagcggcaactccttcctctacgacttccaggtccctgaccaggctggcaccttctggtatcacagccacctttcgacccagtactgcgacggtctccgggggcctctcgttgtgtacgaccccaatgacccacacgctgccctctatgatatcgacgatgataacaccgttattactttgactgactggtaccatactgcggccaggctcggacctcgtttcccgctgggagcagatgccactctcatcaacggcctgggccgcagcccagccacgccgaccgccaacctaactgtcatcaacgttactcagggcaagcgctaccgcttccgcctcgtgtcgatctcttgcgacccgaactatgtgttcagcatcgacaaccacacgatgagcgtcattgagacggacactgtcaacactcaaccgctcacggtcgatagcattcagatctacgccgcccagcgctactcctttgtgctcaccgccaaccagtccgtggataactactggatccgggcaaaccccaacttcggtaacgtcggcttcacggatgctatcaactcggccatcctccgctatgacggtgctcccgacgctgagccctccgctaccactgcaccgacgttgaccaacccgctggttgaggcgaaccttcacccgcttgcttcgatgcccgtgcccggatcccctgtgtctggcggtgtggacaaggccattaacttcgtcttcaacttcaacggcacgaacttctccatcaacaacgcgactttcgttccgcccaccgttccggtgctgctccagatcatgagcggcgccaacaccgcccaagacctcctgccctctggcagcgtgtacacactcccgtccaacgctaccattgagctgtccttccctgcgacgagcaacgcccccggcgctcctcaccccttccacttgcacggtcacgtcttcgccgttgtccgcagcgctggcagcaccgtctacaactacgacaaccccatctggcgcgacgtcgtcagcaccggcacccctgcagcgggcgacaacgtcaccatccgcttccagaccaacaaccctggtccctggttcctccactgtcacatcgacttccacctcgacgccggctttgccgtggtcatggctgaggaccctgttgacactccgacggcggatcccgttccccaggcgtggtccgatctctgcccgacatacgacgcgctttccgtcgacgaccagtga

SEQ ID NO: 58 - protein, 521 aa, Lentinus sp.
MAKFQSLLSYTVLSFVAAAYAAIGPVADLTISNAQVSPDGFLRDAVVTNGLVPGPLITGNKGDRFQLNVIDQMTNHTMLKTTSIHWHGFFQKGTNWADGPAFVNQCPIASGNSFLYDFQVPDQAGTFWYHSHLSTQYCDGLRGPLVVYDPNDPHAALYDIDDDNTVITLTDWYHTAARLGPRFPLGADATLINGLGRSPATPTANLTVINVTQGKRYRFRLVSISCDPNYVFSIDNHTMSVIETDTVNTQPLTVDSIQIYAAQRYSFVLTANQSVDNYWIRANPNFGNVGFTDAINSAILRYDGAPDAEPSATTAPTLTNPLVEANLHPLASMPVPGSPVSGGVDKAINFVFNFNGTNFSINNATFVPPTVPVLLQIMSGANTAQDLLPSGSVYTLPSNATIELSFPATSNAPGAPHPFHLHGHVFAVVRSAGSTVYNYDNPIWRDVVSTGTPAAGDNVTIRFQTNNPGPWFLHCHIDFHLDAGFAVVMAEDPVDTPTADPVPQAWSDLCPTYDALSVDDQ

SEQ ID NO: 59 - DNA, 1575 bp, Trametes sp.
atgggcagacttcagcgtttttcagccttcgttcccctcacactctccttcatatctcaagcgtccgctgcaataggacctgtcacggacttgaccatctccgatgctgacatctcccccgatggtttcactcgtgccgccgtggtgatgaatgaccaattccccggacccttgatcgctggaaacaagggagacaacttccaaatcaatgtcatcgacaatctctccaatagtacaatgctcacttccaccactatccactggcacggcttcttccagaaaggcactaattgggcggacggtgcggcattcgtcaatcaatgtccgatctcggccggcaattcgttcttgtacgacttcacggcgacggaccaagccggcacattctggtatcacagtcacttgtcgacgcagtactgtgatggcctgcgtggtcccatggttgtctatgatcccgacgatccacatgcctccctgtacgatgtggacgacgattcaactgtcattacgctctcggactggtaccacactgccgcgcgtctcggcgctcgtttccctgctggggccgactcaactctcattaacggtttgggccgtgcggcaggcggcgatgcggacgccgctctcgcagtattcaacgttacccaaggctcgcgttaccgcttccgcctggtttccctgtcatgcgacccgaacttcaacttcaccatccaagatcacaacatgacgatcatcgaggttgatggggtcaacgtcgagcccgtcactgtcgactcgatccagattttcgccgggcagagatactccttcgtgctcaccgcggatcaagatatcggtaactactggatccaggccgttcctaacaccggtacagtcaccaccgatggcggcgttaactctgccattctgcgttacgacacggcggacccgatcgaacccgacgccgcagaccccaccagcagtatcccgctcgtggagacagacctcgtcccgctggagaacctcgcagcgcccggagatcccaccgtcggtggtgttgacctggcgatgaacctggagttcgactttaatggcacgtggttctttatcaacggcgagccattcgttcctcctagtgtccctgttttgctgcaaatcatgagtggcgcgcagtctgctgcggaccttctcccgagcggaagcgtatacacgctccccgccaactctaccatcgagatttccttccctatgaacactacagcagcgcccggtgcgccgcatccgttccaccttcacgggcacacgttctacgtcgtgcgcagcgcgggcagcaccgaatacaactacgtgaacccaccccagcgcgacaccgtcagcacgggcaccgacggagacaatgtcaccatccggttcacgacgaacaaccccggcccgtggttcctccactgccacatcgactttcacctcgacgccggcttcgccatcgtgctcagcgaggacactccggacgctgcttcggccaacacgccctcctctgcgtgggatgatctttgccccacttataacaccgactatcccgacggtctcgggcgctga

SEQ ID NO: 60 - protein, 524 aa, Trametes sp.
MGRLQRFSAFVPLTLSFISQASAAIGPVTDLTISDADISPDGFTRAAVVMNDQFPGPLIAGNKGDNFQINVIDNLSNSTMLTSTTIHWHGFFQKGTNWADGAAFVNQCPISAGNSFLYDFTATDQAGTFWYHSHLSTQYCDGLRGPMVVYDPDDPHASLYDVDDDSTVITLSDWYHTAARLGARFPAGADSTLINGLGRAAGGDADAALAVFNVTQGSRYRFRLVSLSCDPNFNFTIQDHNMTIIEVDGVNVEPVTVDSIQIFAGQRYSFVLTADQDIGNYWIQAVPNTGTVTTDGGVNSAILRYDTADPIEPDAADPTSSIPLVETDLVPLENLAAPGDPTVGGVDLAMNLEFDFNGTWFFINGEPFVPPSVPVLLQIMSGAQSAADLLPSGSVYTLPANSTIEISFPMNTTAAPGAPHPFHLHGHTFYVVRSAGSTEYNYVNPPQRDTVSTGTDGDNVTIRFTTNNPGPWFLHCHIDFHLDAGFAIVLSEDTPDAASANTPSSAWDDLCPTYNTDYPDGLGR

SEQ ID NO: 61 - DNA, 1554 bp, Basidiomycete PM1
atggccaagttccaatctctcctcaccttcatcaccctctcgctcgttgcctcagtgtacgctagcattgggccagtcgcagacctcaccatctccaacggtgctgtcagtcccgatggtttctctcggcaggccatcctggtcaacgacgtcttccccagtcccctcattacggggaacaagggtgatcgtttccaactcaatgtcatcgacaacatgaccaaccacaccatgttgaagtccaccagtatccattggcacggcttcttccaacacggcaccaactgggccgacggccccgccttcgtgaaccagtgcccgatttctaccgggcatgcgttcctttacgacttccaggtccctgaccaagctggtactttctggtaccacagtcacttgtccactcaatactgtgacggtctcaggggtccgattgttgtctatgaccctcaagatccccacaagagcctttacgatgttgatgacgactccactgtaatcactctcgcggattggtaccacttggctgccaaagtcggcccggcggtcccgactgccgatgcgactcttatcaacggcctcggtcgcagcatcaacacgctcaacgccgatttggctgtcatcacggtcacgaagggcaagcgctatcgcttccgcctggtgtcgctgtcatgcgacccgaatcacacgttcagcattgatggtcactctctgaccgtcatcgaggcggacagcgtgaatctcaagccccagactgtcgactccatccagatcttcgctgcccagcggtactcgtttgtgctcaacgcagatcaggatgtggacaactactggatccgtgcccttcccaactccgggaccaggaacttcgacggcggcgttaactccgccatccttcgctacgacggtgctgcgcccgttgagcccaccacgacccagacgccgtcgacgcagcctttggtggagtccgccctgaccactctcgaaggcaccgctgcgcccggcaacccgacccctggcggtgtcgacctggctctcaacatggctttcggctttgccggcggcaggttcaccatcaacggcgcgagcttcaccccgcccaccgtccccgtcctcctgcagatcctgagcggcgcgcagtcggcgcaggacctcctcccctctggaagtgtatactcgctccctgcgaacgcggacattgagatctccctccccgccacctccgccgcccccggcttcccgcaccccttccacttgcacgggcacaccttcgccgtcgtgcgcagcgccggctcgtcgacgtacaactacgcgaacccggtctaccgcgacgtcgtcagcacgggctcgcccggggacaacgtcacgatccggttcaggacggacaaccccggcccgtggttcctccactgccacatcgacttccacctcgaggctgggttcgcggtcgtcatggccgaggacattcccgacgtcgccgctacgaacccggtcccgcaagcatggtcggatctgtgcccgacctatgatgcgctctcgcctgacgaccagtga

SEQ ID NO: 62 - protein, 517 aa, Basidiomycete PM1
MAKFQSLLTFITLSLVASVYASIGPVADLTISNGAVSPDGFSRQAILVNDVFPSPLITGNKGDRFQLNVIDNMTNHTMLKSTSIHWHGFFQHGTNWADGPAFVNQCPISTGHAFLYDFQVPDQAGTFWYHSHLSTQYCDGLRGPIVVYDPQDPHKSLYDVDDDSTVITLADWYHLAAKVGPAVPTADATLINGLGRSINTLNADLAVITVTKGKRYRFRLVSLSCDPNHTFSIDGHSLTVIEADSVNLKPQTVDSIQIFAAQRYSFVLNADQDVDNYWIRALPNSGTRNFDGGVNSAILRYDGAAPVEPTTTQTPSTQPLVESALTTLEGTAAPGNPTPGGVDLALNMAFGFAGGRFTINGASFTPPTVPVLLQILSGAQSAQDLLPSGSVYSLPANADIEISLPATSAAPGFPHPFHLHGHTFAVVRSAGSSTYNYANPVYRDVVSTGSPGDNVTIRFRTDNPGPWFLHCHIDFHLEAGFAVVMAEDIPDVAATNPVPQAWSDLCPTYDALSPDDQ

SEQ ID NO: 63 - DNA, 1620 bp, Coprinopsis cinerea
atggtcaagaacctcctctcgttcgcccttctggcgattagcgttgccaacgctcagatcgtcaattcggtcgataccatgaccctcaccaacgcgaacgtcagtcccgacggtttcactcgagctggtatcctcgtcaatggagttcatggacctcttattcgaggtggaaagaacgacaactttgagctcaacgtcgttaacgacttggacaaccccactatgcttcggcctaccagtatccattggcacggtctcttccaacgagggaccaactgggctgatggtgcagatggtgtcaaccagtgcccgatctctccaggccatgctttcctctacaagttcactccagctggccacgctggtactttctggtaccattcccactttggcacccaatactgcgatggtctccgtggtccaatggtcatttacgacgacaatgacccacacgctgccctctacgacgaggatgacgagaacaccatcattaccctcgccgattggtaccatatccccgctccctccattcagggtgctgcccagcctgacgctacgctcatcaacggtaagggtcgctacgtgggcggcccagctgccgagctttcgatcgtcaatgtcgagcaagggaagaagtaccgaatgcgtttgatctcgctgtcctgcgaccccaactggcagttctccattgacggacatgagttgacgatcattgaagtcgatggtcagcttactgagccgcatacggttgatcgtctccagatcttcactggtcaaaggtactccttcgttctcgacgccaaccagccggtggacaactactggatccgtgctcaacccaacaagggtcgaaacggacttgctggtaccttcgccaacggtgtcaactcggccatccttcgctatgccggcgctgccaacgctgatccaaccacctccgccaaccccaaccccgcccaactcaacgaagccgacctccatgctctcatcgaccccgctgctcccggtatccccactccgggcgctgcagacgtcaacctccgattccaattgggcttcagcggcggtcgattcacgattaacggaaccgcatacgagagtccaagcgttcctacgctcttgcagattatgagtggtgcgcagagtgcgaacgacttgctccctgctggatcggtgtatgagttgcccaggaaccaagttgttgagcttgttgttcctgctggtgtcctcggtggtcctcatcctttccatctccacggtcatgcgttcagtgtcgtcaggagtgcaggcagcagcacctacaactttgtcaaccccgtcaagcgcgatgttgttagtcttggtgttactggagacgaagttaccattcgattcgtcaccgataacccaggcccgtggttcttccactgccacattgaattccatctcatgaacggcttggcgatcgtctttgctgaagacatggcgaacacggttgatgctaacaacccacctgtcgagtgggcccagctttgcgagatttacgatgacctgccgcctgaggcgacctcgattcaaaccgttgtgcgtcgcgctgagcccaccggcttttcggccaagttccgcagggagggcttgtag

SEQ ID NO: 64 - protein, 539 aa, Coprinopsis cinerea
MVKNLLSFALLAISVANAQIVNSVDTMTLTNANVSPDGFTRAGILVNGVHGPLIRGGKNDNFELNVVNDLDNPTMLRPTSIHWHGLFQRGTNWADGADGVNQCPISPGHAFLYKFTPAGHAGTFWYHSHFGTQYCDGLRGPMVIYDDNDPHAALYDEDDENTIITLADWYHIPAPSIQGAAQPDATLINGKGRYVGGPAAELSIVNVEQGKKYRMRLISLSCDPNWQFSIDGHELTIIEVDGQLTEPHTVDRLQIFTGQRYSFVLDANQPVDNYWIRAQPNKGRNGLAGTFANGVNSAILRYAGAANADPTTSANPNPAQLNEADLHALIDPAAPGIPTPGAADVNLRFQLGFSGGRFTINGTAYESPSVPTLLQIMSGAQSANDLLPAGSVYELPRNQVVELVVPAGVLGGPHPFHLHGHAFSVVRSAGSSTYNFVNPVKRDVVSLGVTGDEVTIRFVTDNPGPWFFHCHIEFHLMNGLAIVFAEDMANTVDANNPPVEWAQLCEIYDDLPPEATSIQTVVRRAEPTGFSAKFRREGL

SEQ ID NO: 65 - DNA, 1602 bp, Pleurotus ostreatus
atgtttccaggcgcacggattcttgctacgcttaccttggctcttcatcttttacatgggactcatgctgccatcgggcccactggcaacatgtacatcgtcaacgaggacgtctctcctgatggattcgctcgttcggcggttgtcgctcgctcggtgcccgctacagatccgacgcctgcgacagtatccattcctggcgttctcgttcaaggaaacaagggcgataacttccagctgaacgtcgtcaatcaattgtcggacacgaccatgttgaagacgaccagtatccattggcacggtttcttccaagccggatcttcgtgggctgatggtcccgctttcgtgacccaatgccccgtcgcctctggggatagtttcctgtacaatttcaatgtcccagaccaagctggaacgttttggtatcactcgcatctttccacccaatattgtgacggcctcagaggaccattcgtggtatacgacccctcggatccgcacttgagtttatacgatattgacaacgccgacacggtcattacgcttgaggattggtatcatatcgtggctccccaaaacgcggcaatcccaactccggatagtaccctcatcaatggtaaaggtcgttatgccgggggccctacctctcctttgtccatcatcaacgtcgaaagcaacaagcgctatcgtttcagacttgtctcaatgtcttgtgaccccaatttcacgttctcgatcgacggtcactctttgctcgtcattgaagcagatgctgtcaacattgttcccatcaccgtggatagtattcagatcttcgctggccaacgctactccttcgtcttgactgctgatcaaaccgttggcaactactggattcgcgcgaatcctaacttgggatcgactggcttcgatggtggtatcaattccgctattcttcggtatgctggtgccactgaggatgaccccaccacaacctcgtcgacgagcaccccattgctggagaccaaccttgttccgcttgagaatcctggtgctcctggcccagccgtgcctggtggagcagacatcaacatcaatctcgctatggccttcgacttcactaacttcgaattgactatcaacggcgttcctttcatcccacccactgcccctgtccttcttcaaattctctcaggagcctcctctgctgcctcgctgcttccttctggtagtatttacgcgctggagcctaataaggttgttgaaatctcgatgcctgcgctggctgtcgggggaccccatccattccatctccacggccacaccttcgacgttattaggagtgcgggttccactacatacaactttgacactcctgcgcgccgcgacgtagtcaacactggcactggcgcgaacgacaacgtcactattcgcttcgtgaccgacaacccagggccgtggttcctccactgtcacattgattggcatctcgaaattggtctcgctgtcgttttcgccgaagacgtgacatccatttcggccccacctgccgcgtgggacgacttgtgccccatctatgacgcattgagcgacaacgacaaaggaggcatcgttccgtcctaa

SEQ ID NO: 66 - protein, 533 aa, Pleurotus ostreatus
MFPGARILATLTLALHLLHGTHAAIGPTGNMYIVNEDVSPDGFARSAVVARSVPATDPTPATVSIPGVLVQGNKGDNFQLNVVNQLSDTTMLKTTSIHWHGFFQAGSSWADGPAFVTQCPVASGDSFLYNFNVPDQAGTFWYHSHLSTQYCDGLRGPFVVYDPSDPHLSLYDIDNADTVITLEDWYHIVAPQNAAIPTPDSTLINGKGRYAGGPTSPLSIINVESNKRYRFRLVSMSCDPNFTFSIDGHSLLVIEADAVNIVPITVDSIQIFAGQRYSFVLTADQTVGNYWIRANPNLGSTGFDGGINSAILRYAGATEDDPTTTSSTSTPLLETNLVPLENPGAPGPAVPGGADININLAMAFDFTNFELTINGVPFIPPTAPVLLQILSGASSAASLLPSGSIYALEPNKVVEISMPALAVGGPHPFHLHGHTFDVIRSAGSTTYNFDTPARRDVVNTGTGANDNVTIRFVTDNPGPWFLHCHIDWHLEIGLAVVFAEDVTSISAPPAAWDDLCPIYDALSDNDKGGIVPS

SEQ ID NO: 67 - DNA, 1596 bp, Thanatephorus cucumeris
atgctttctagcattaccctcctacctttgcttgctgcggtttcaacccccgcctttgctgccgtccgcaactacaagttcgacatcaagaacgtcaatgtcgctcccgatggctttcagcgtcctatcgtctccgtcaacggtctagttcctggcacgttgatcacggccaacaagggcgacaccttgcgcattaatgtcacgaatcaactcacggaccctagtatgcgtcgtgccacaacgattcattggcatggattgttccaagctactaccgccgacgaggatggccccgcattcgtcacgcaatgccctattgcgcaaaatttgtcctatacatacgagatcccgttgcacggccaaacaggaaccatgtggtatcacgcccatcttgcgagtcaatatgtcgatggattgcgaggccctttggtcatctatgatccaaacgacccacacaagtcgcgctacgacgtggatgatgcgagcacagtagtcatgcttgaggactggtaccatactccggcacccgttctagaaaagcaaatgttctcgactaataacaccgctctgctctctcctgttccggactcgggtcttatcaatggcaaagggcgctatgtgggcggtcccgcagttccccggtcagtaatcaacgtaaaacgtgggaaacgatatcgcttgcgcgtaatcaacgcttctgctatcgggtcgtttaccttttcgatcgaaggacatcgtctgactgtcattgaggccgatgggatcccgcaccagcccttgcctgttgatagcttccagatttacgctggacaacgctactctgtcatcgttgaagccaaccaaaccgctgccaattactggattcgcgcaccaatgaccgttgcaggagcaggaaccaacgcaaacttggaccccaccaatgtctttgccgtgttgcactacgagggagcacccaacgccgaacccacgacggaacaaggcagtgctatcggtactgcactcgttgaagagaacctccatgcgctcatcaaccctggcgctccgggcggctccgctcccgcagacgtttccctcaatctcgcaattgggcgcagtacagttgatgggattcttaggttcacatttaataacatcaagtacgaggctccttcgttgcccacgctcttgaagattttggcaaataatgcgagcaatgacgccgatttcacgccaaatgagcacactatcgtattgccacacaataaagttatcggagctcaacatcaccgaggtgcagaccaccctatccatctccacggccatgtgtttgacattgtcaaatcgctcggtggtaccccgaactatgtcaacccgcctcgcagggatgtagttcgtgtcggaggcaccggtgtggtactccgattcaaggccgataacccaggcccatggtttgttcactgccacattgactgcacttggaggctgggctcgcacttgtctttgccgaggcccccagccagattcgccagggtgtccagtcggtccagcccaacaatgcctggaaccagctctgccccaagtacgcggctcttcctcccgatttgcagtaaatggtga

SEQ ID NO: 68 - protein, 531 aa, Thanatephorus cucumeris
MLSSITLLPLLAAVSTPAFAAVRNYKFDIKNVNVAPDGFQRPIVSVNGLVPGTLITANKGDTLRINVTNQLTDPSMRRATTIHWHGLFQATTADEDGPAFVTQCPIAQNLSYTYEIPLHGQTGTMWYHAHLASQYVDGLRGPLVIYDPNDPHKSRYDVDDASTVVMLEDWYHTPAPVLEKQMFSTNNTALLSPVPDSGLINGKGRYVGGPAVPRSVINVKRGKRYRLRVINASAIGSFTFSIEGHRLTVIEADGIPHQPLPVDSFQIYAGQRYSVIVEANQTAANYWIRAPMTVAGAGTNANLDPTNVFAVLHYEGAPNAEPTTEQGSAIGTALVEENLHALINPGAPGGSAPADVSLNLAIGRSTVDGILRFTFNNIKYEAPSLPTLLKILANNASNDADFTPNEHTIVLPHNKVIGAQHHRGADHPIHLHGHVFDIVKSLGGTPNYVNPPRRDVVRVGGTGVVLRFKADNPGPWFVHCHIDCTWRLGSHLSLPRPPARFARVSSRSSPTMPGTSSAPSTRLFLPICSKW

SEQ ID NO: 69 - DNA, 1557 bp, Volvariella volvacea
atgcaatctttgctcaacacactcaccgccatggtgaccgtggtgggatggggtgctaactttgctgcagccgcattgagctcgcatacgttgacacttaccaatggcttcgcctcccccgatggccactctcgcgaagtggttctggtcaatggggggctgttccaagctgtcatcgcgggtaacaagggcgatgacttcgagatcgaagtagacaaccaattgaccgttgagattttacgcaagagtacctctattcactggcacggactgttccaacgcggaagtgcatgggcagatggtcctgccttcgtcactcagtgcccaattgctcctggaaataccttcacctacgagttcacgcccaccgatgaagttgggacattctggtatcattcccatctcgatgcgcaatattgtgatggactcagaggaccctttgtcatctatgaccccaacgaccctcatctcgccctctacgatgttgacgatgaggataccatcattactctggctgattggtaccacactgcggctgagttactcaccggtgtagttattcctgactcggctcttatcaatggtttgggtcgcacatccacgacaactacttcacctctcgctgtgataaacgttgtacaaggaaccaagtatcgcatgaggctgatttcgatctcttgcgatccaaacaactatatattctccattgaagatcatgagatgacagtaattgaagcggatggtattagtgtggatcctgttactgtgacatcattgcagattttcgttggccaacgatactcctttatccttcacgcaaaccaacccgttgataactactggatccgtgcaaaccccaacctaggaccaaccggattttctggtggcatcaatagtgcaattttgcgctaccaaggagcaccagttgcagaccccaccggtccaggacttcaggatgcactcaaccgtctggcagaaactgacttgcaccccatcgtcaaccctggtgctcctgacccagtagacattgacttggttatcaatattggattttctgctggtttattcaacatcgatggtacttcatacgtatctcccgatgttccatctctccttcagatccttaacggtgttcccgttagctcgctcttgcctagtggttcatacatcgaattgccacctaataaggtagtgcagctttcattcccagtgattgctggccaaggttccgccattggtgctcctcatcccatccatcttcacggccacgccttcgacgtcattcgtagcgccggatcttcaacctataaccttgtcgatcctgtccgtcgggatgtcgtttctataggtacacctggcgataacgttacaatccgcttcgtcaccgataatgcaggcccttggtacttgcactgccatattgagtggcacctccgcgctgggctgggtgtcatttttgctgaagatgctgcaggaagtctacttcaacctgcacctccaacggcttggggtgatctttgcgatatttacgatctcttgccccctgaggatcagtaa

SEQ ID NO: 70 - protein, 518 aa, Volvariella volvacea
MQSLLNTLTAMVTVVGWGANFAAAALSSHTLTLTNGFASPDGHSREVVLVNGGLFQAVIAGNKGDDFEIEVDNQLTVEILRKSTSIHWHGLFQRGSAWADGPAFVTQCPIAPGNTFTYEFTPTDEVGTFWYHSHLDAQYCDGLRGPFVIYDPNDPHLALYDVDDEDTIITLADWYHTAAELLTGVVIPDSALINGLGRTSTTTTSPLAVINVVQGTKYRMRLISISCDPNNYIFSIEDHEMTVIEADGISVDPVTVTSLQIFVGQRYSFILHANQPVDNYWIRANPNLGPTGFSGGINSAILRYQGAPVADPTGPGLQDALNRLAETDLHPIVNPGAPDPVDIDLVINIGFSAGLFNIDGTSYVSPDVPSLLQILNGVPVSSLLPSGSYIELPPNKVVQLSFPVIAGQGSAIGAPHPIHLHGHAFDVIRSAGSSTYNLVDPVRRDVVSIGTPGDNVTIRFVTDNAGPWYLHCHIEWHLRAGLGVIFAEDAAGSLLQPAPPTAWGDLCDIYDLLPPEDQ

SEQ ID NO: 71 - DNA, 59 bp, Artificial Sequence
  Artificial DNA Primer
tcctctatatacacaactggggatccaccatgtcgaggtttcactctcttctcgctttc

SEQ ID NO: 72 - DNA, 49 bp, Artificial Sequence
  Artificial DNA Primer
tctagatctcgagctcgctagagtcgacctactggtcgctcgggtcgag

SEQ ID NO: 73 - DNA, 31 bp, Artificial Sequence
  Artificial DNA Primer
catggtggatccccagttgtgtatatagagg

SEQ ID NO: 74 - DNA, 27 bp, Artificial Sequence
  Artificial DNA Primer
taggtcgactctagcgagctcgagatc

SEQ ID NO: 75 - DNA, 36 bp, Artificial Sequence
  Artificial DNA Primer
acatgtctttgataagctagcgggccgcatcatgta

SEQ ID NO: 76 - DNA, 36 bp, Artificial Sequence
  Artificial DNA Primer
tacatgatgcggcccgctagcttatcaaagacatgt

SEQ ID NO: 77 - DNA, 41 bp, Artificial Sequence
  Artificial DNA Primer
ttaatcgccttgcagcacaccgcttcctcgctcactgactc

SEQ ID NO: 78 - DNA, 47 bp, Artificial Sequence
  Artificial DNA Primer
acaataaccctgataaatgcggaacaacactcaaccctatctcggtc

SEQ ID NO: 79 - DNA, 53 bp, Artificial Sequence
  Artificial DNA Primer
agatagggttgagtgttgttccgcatttatcagggttattgtctcatgagcgg

SEQ ID NO: 80 - DNA, 42 bp, Artificial Sequence
  Artificial DNA Primer
ttctacacgaaggaaagaggaggagagagttgaacctggacg

SEQ ID NO: 81 - DNA, 47 bp, Artificial Sequence
  Artificial DNA Primer
aggttcaactctctcctcctctttccttcgtgtagaagaccagacag

SEQ ID NO: 82 - DNA, 43 bp, Artificial Sequence
  Artificial DNA Primer
tcagtgagcgaggaagcggtgtgctgcaaggcgattaagttgg

SEQ ID NO: 83 - DNA, 40 bp, Artificial Sequence
  Artificial DNA Primer
tcaaccgcggactgcgcaccatgtcgaggtttcactctct

SEQ ID NO: 84 - DNA, 40 bp, Artificial Sequence
  Artificial DNA Primer
ggctttcgccacggagcttactactggtcgctcgggtcga

SEQ ID NO: 85 - DNA, 27 bp, Artificial Sequence
  Artificial DNA Primer
ctggccgtagagcttaaagtatgtccc

SEQ ID NO: 86 - DNA, 30 bp, Artificial Sequence
  Artificial DNA Primer
cggtcgattacaatcacatgacttggcttc

SEQ ID NO: 87 - DNA, 11101 bp, Artificial Sequence
  Artificial DNA Sequence
ttgaagttcctattccgagttcctattctctagaaagtataggaacttcagtacccgggtataagctagcttccgttaaattgccgtcgtcagccgttaaattaccgattaatcccgataaatttccgagatctccgttaaattgccgttcgcagccgttaaattaccggggacgaccgataaatttccgcgatgaattcatggtgttttgatcattttaaatttttatatggcgggtggtgggcaactcgcttgcgcgggcaactcgcttaccgattacgttagggctgatatttacgtaaaaatcgtcaagggatgcaagaccaaaccgttaaatttccggagtcaacagcatccaagcccaagtccttcacggagaaaccccagcgtccacatcacgagcgaaggaccacctctaggcatcggacgcaccatccaattagaagcagcaaagcgaaacagcccaagaaaaaggtcggcccgtcggccttttctgcaacgctgatcacgggcagcgatccaaccaacaccctccagagtgactaggggcggaaatttatcgggattaatttccactcaaccacaaatcacagtcgtccccggtaatttaacggctgcagacggcaatttaacggcttctgcgaatcgcttggattccccgcccctggccgtagagcttaaagtatgtcccttgtcgatgcgatgtatcacaacatataaatactggcaagggatgccatgcttggagtttccaactcaatttacctctatccacacttctcttccttcctcaatcctctatatacacaactggggatccaccatgttctcggcaggccacaagattaagggtacagtcgtcctcatgcctaaaaacgagttggaagtgaaccccgatggctccgcagtcgataacctcaacgcattcctcggacgttcggtgtcgctccagctcatctccgcgaccaaagccgacgcccacggtaagggaaaggtgggcaaggacacgttcttggaaggtatcaacacttcgctccctaccttgggagcaggagagtccgcattcaacattcacttcgagtgggacggttcgatgggcattcccggagcgttctatatcaagaactatatgcaggtggagttcttcttgaagtccttgaccttggaggcaatctcgaaccagggtaccatccgtttcgtgtgtaactcgtgggtctacaacaccaagctctacaaatccgtgcggatcttcttcgcgaaccacacttacgtcccttcggagacacctgcccctttggtgtcgtaccgcgaggaggaattgaagtccctccgtggtaacggtactggagaaaggaaggagtatgataggatctacgactacgacgtctataacgatttgggtaaccccgacaaatcggaaaagttggcacgtcctgtgttgggaggctcctccaccttcccctaccctcgacgcggccgcacgggacgcggtcccactgtcaccgatccgaacacagagaagcagggcgaagtcttctacgtgcccagggacgaaaacctcggccacttgaagtcgaaggatgcattggagattggaaccaagtccctctcccagatcgtccagcctgcattcgaatcggcgttcgatttgaaatcgacgcccatcgagttccactcgttccaggacgtccatgacttgtatgaaggtggtatcaaattgcctcgggacgtcatctccaccattatccccctccccgtgatcaaggaattgtaccgcaccgacggccagcatattctcaaattcccccagccgcacgtcgtccaggtctcgcagtccgcatggatgacagatgaggaattcgcgagggaaatgattgcaggtgtcaacccgtgtgtcatccgaggcttggaggagttccctcctaagtccaacctcgatcctgccatctatggagaccagtcctccaagattacagccgattccctcgatctcgacggttatactatggatgaagcactcggttccaggcgattgttcatgctcgattatcatgatatcttcatgccctatgtgcgccagatcaaccagttgaactcggcaaaaacatatgcaacgaggacgatcctcttcctccgagaagacggcacactcaagcctgtggcaatcgagctctcgctcccccattccgcaggcgatctctccgcagccgtgtcgcaggtggtgttgcctgcaaaagaaggagtggagtcgaccatctggctcttggccaaagcatatgtgattgtgaacgattcctgttatcaccagctcatgtcgcattggctcaacactcacgcggcaatggaacccttcgtgatcgccacgcaccggcacctctcggtgctccacccgatctacaagctcctcactccccactaccgtaacaacatgaacattaacgccttggcacggcagtcgttgatcaacgcgaacggcatcattgagacaacgttcctcccctccaagtactccgtcgaaatgtcgtccgcagtctacaaaaactgggtcttcaccgaccaggcgttgcctgccgacttgatcaaacgaggcgtcgcaatcaaagatccctccactcctcatggcgtccgcctcttgatcgaggactacccctacgcagcggacggattggaaatctgggcagccatcaagacctgggtgcaggaatacgtccctttgtactatgcgagggacgatgatgtcaaaaacgactcggaactccagcattggtggaaggaggcagtggaaaagggccatggagatctcaaggataaaccctggtggcctaagctccagaccttggaggacctcgtcgaagtgtgtttgatcattatctggatcgcatccgcgttgcatgcagccgtgaacttcggacagtatccctatggaggcctcatcatgaaccgtcccaccgcatccaggaggctcctccccgaaaaaggaacacccgaatacgaagaaatgatcaacaaccacgaaaaggcatacctccggaccatcacttccaaactcccgaccttgatctcgctctccgtgatcgagattttgtcgacacatgcgtcggacgaggtctatttgggtcagcgggataacccgcactggacatccgattccaaggccctccaggcgttccagaagttcggcaacaagctcaaggagatcgaggagaaactcgtgaggcggaacaacgacccttccctccagggaaaccggttgggacctgtccagctcccgtatacgttgctctacccctcctcggaagaaggcctcactttcaggggtatccccaactcgatttccatctgactcgagatctagagggtgactgacacctggcggtagacaatcaatccatttcgctatagttaaaggatggggatgagggcaattggttatatgatcatgtatgtagtgggtgtgcataatagtagtgaaatggaagccaagtcatgtgattgtaatcgaccgacggaattgaggatatccggaaatacagacaccgtgaaagccatggtctttccttcgtgtagaagaccagacagacagtccctgatttacccttgcacaaagcactagaaaattagcattccatccttctctgcttgctctgctgatatcactgtcattcaatgcatagccatgagctcatcttagatccaagcacgtaattccatagccgaggtccacagtggagcagcaacattccccatcattgctttccccaggggcctcccaacgactaaatcaagagtatatctctaccgtccaatagatcgtcttcgcttcaaaatctttgacaattccaagagggtccccatccatcaaacccagttcaataatagccgagatgcatggtggagtcaattaggcagtattgctggaatgtcggggccagttggccgggtggtcattggccgcctgtgatgccatctgccactaaatccgatcattgatccaccgcccacgaggcgcgtctttgctttttgcgcggcgtccaggttcaactctctcttaattaaatagcgacaagccgaacggcaccggcaggtacaatggttcgctgtacttgcttgcgcaagcgggtctttggggattgagcgcatttggtgttgcaaaggatttgatgtaaatgtagtcgacatcttagcacagaggggagagttgataaaatgtggtctgtttgaatgatagtcgggttcgtgacctatattcgtgatagtggagataggtctgcgcctatcttatcgggccggagcaaaaattccaccgcagcggggtgagttttcgttatacagccatcccacttccagcttcaaattgtcagtttaatccagcccaattcaatcattggagaaccggttttatgtcttcgaagtcccacctcccctacgcaattcgcgcaaccaaccatcccaaccctttaacatctaaactcttctccatcgccgaggagaagaaaaccaacgtcaccgtctccgcagacgttactacttccgccgagctcctcgatcttgctgaccgcctaggcccctatatcgcagttctgaaaacccacatcgacatcctcaccgatctcaccccgtcgaccctttcctcgctccaatccctcgcgacaaagcacaacttcctcatctttgaggaccgcaagttcatcgacatcggcaacaccgtgcaaaagcagtaccacggtggcgctctccgcatctccgaatgggcacacatcatcaactgcgccatcctgccgggcgaagggatcgtcgaggccctcgcacagacaaccaagtctcctgactttaaagacgcgaatcaacgaggtctcctgattcttgccgagatgacgagtaagggatctcttgcgacaggggagtacacggcacgctcggttgagtacgcgcggaagtataaggggtttgtgatgggattcgtgagtacaagggcgttgagtgaggtgctgcccgaacagaaagaggagagcgaggattttgtcgtctttacgactggggtgaatctgtcggataagggggataagctggggcagcagtatcagacacctgggtcggcggttgggcgaggtgcggactttatcattgcgggtaggggcatctataaggcggacgatccagtcgaggcggttcagaggtaccgggaggaaggctggaaagcttacgagaaaagagttggactttgagggtgactgacacctggcggtagacaatcaatccatttcgctatagttaaaggatggggatgagggcaattggttatatgatcatgtatgtagtgggtgtgcataatagtagtgaaatggaagccaagtcatgtgattgtaatcgaccgacggaattgaggatatccggaaatacagacaccgtgaaagccatggtctttccttcgtgtagaagaccagacagacagtccctgatttacccttgcacaaagcactagaaaattagcattccatccttctctgcttgctctgctgatatcactgtcattcaatgcatagccatgagctcatcttagatccaagcacgtaattccatagccgaggtccacagtggagcagcaacattccccatcattgctttccccaggggcctcccaacgactaaatcaagagtatatctctaccgtccaatagatcgtcttcgcttcaaaatctttgacaattccaagagggtccccatccatcaaacccagttcaataatagccgagatgcatggtggagtcaattaggcagtattgctggaatgtcggggccagttggccgggtggtcattggccgcctgtgatgccatctgccactaaatccgatcattgatccaccgcccacgaggcgcgtctttgctttttgcgcggcgtccaggttcaactctctcctctaggttgaagttcctattccgagttcctattcttcaaatagtataggaacttcaactagctagtgcatgcgtacgattttgacatttgctccattgtcgaggatggatggaacgagcggcgtgcgccacgaaagtgaggctattgcctatcagctctttgctacattccggaaacaaacatccctttttgtgaattatctacgcaacttagatggcgtgaacgcatcttcaaagtctttcggcaggtccggcacgacttttgcatccagagaagcgcctacatgtgtattcgaccacctcctagcgcgcttggatatgaggaaatattactgagagtcgaaaacaagctccaccgcaccagctcttcttggagttttatattaaagaatattcccagctcgttgtattattctttttctaccgtgctaatgtatcaaggactttggtacctattaacgttattattcgtgtgctattcccaaacataaccctgtatatgtttcgaacgccgttatgacccatgtcttacatactcattaagtcattcccttggataatctcgactcagatgcggcggttgatgtaggaggagaggtaatcgaggacctcctgggagatgatgccgttccaggcggggtagcggatggagccctcggcggagcccttgagctgctcgatatgctgccactcctcgatggggttggtctcatccttgagggcgatcatctccttggagatgggatcgtaggcgtagtagcgggagactagtgcgaagtaatgatcggggatggcggtgatctgatgggtgtaggtggtgcgggcgacggcggaggcgcgcttatcggaccagttgccgacgacgttggtgagctcggtgaggcccttcatggagaggaaggaggtcatgagatggcggccgatatgggacttggggccgttcttgatggcgaagatggagtagggggcgttcttcttgagggccttgttgtaggagcggacgaggttatccttgaggagctggtactcctgcttgttggaggaggagttgccggtgcggttgacgcgcttgaggacgggctcggagttgcggaggaactcatcgaggtagacgaggggatcgatgcggccgcgggcggagaagaagtagatatggcgggagacggaggtcttggtctcggtgacgaggcactggatgatgacgccgaggtacttgttctggacgagcttgaaggacttgggatcgacgttcttgatatcggagaagcggccgcagttgatgaaggtggcgaggaagaggaactggtagagggtcttggtcttggtgaagcgggaggtgtactcgaaggagttgaggatcttctcggtgatctcccagatggactcgccctcggagaggagggccttgagcatcttcttggaatgggagttgcccttatcggcctcctcggaggactcgaactggagctggagggaggagacgatatcggtgatatcggactgatgcttctggccgtagtaggggatgatggtgaactcccaggcggggatgagcttcttgagggaggcctccaggatggtggccttctgggtcttgtacttgaactggagggacttgttgacgatatcgaaggagagggagttggagatgatggtgttgtaggacatgaaggtggcgcgcttgatggcggtgccgttatgggtgatcatccagcagaggtaggtgagctcggcggcgcagagggcgatcttctcgccggaggggcgctcgaagcgctcgacgaactggcggacgaggaccttggggggggtcttgcagaggatatcgaactggggcatggtgctcagatactacggctgatcgcgtagaggtactgagcaaaacagatgtcagtaaggagaagagttgaatgaatggaagaagagtaggaaaggaggtatgggggaaagatatacgtactgatgcggacgaagagagaaagaaggaaaaaagttgtgggaggggaaggagggggaatccttatatggaggggcaagcgagaaggcgaattagtgggcgggcttaagccctcgaccgccgcccttatcattggacatggaggggtaatgcccccaccacgcatgtgcgggaccgacgcagaatctgcacggcggagtctcttccagactgttgacttttgggcgatgactcttgttgctgcggccttttgggtacaccaacctcgttgatcttgtttccttggttctctttcgctcggagacccgaccatgaccccaccatcagtcactatcctgcctcgtcgataaaaattttttcttccctctgattgttacatagtatgtttccacctttccggtggatttcggacagtcaaactgggcatcaacgcagtggtgggctgcttcgtttgctgcgtgttgtacttgtttgcatttgaaccccgcggtcgttcgagtccttaattggtccgctcccggtcaacacccaagcagctgtggcccggccgagtggcgcctgtctggtccacagtaagcttggcgtaatcatggtcatagctgtttcctgtgtgaaattgttatccgctcacaattccacacaacatacgagccggaagcataaagtgtaaagcctggggtgcctaatgagtgagctaactcacattaattgcgttgcgctcactgcccgctttccagtcgggaaacctgtcgtgccagctgcattaatgaatcggccaacgcgcggggagaggcggtttgcgtattgggcgctcttccgcttcctcgctcactgactcgctgcgctcggtcgttcggctgcggcgagcggtatcagctcactcaaaggcggtaatacggttatccacagaatcaggggataacgcaggaaagaacatgtgagcaaaaggccagcaaaaggccaggaaccgtaaaaaggccgcgttgctggcgtttttccataggctccgcccccctgacgagcatcacaaaaatcgacgctcaagtcagaggtggcgaaacccgacaggactataaagataccaggcgtttccccctggaagctccctcgtgcgctctcctgttccgaccctgccgcttaccggatacctgtccgcctttttcccttcgggaagcgtggcgctttctcatagctcacgctgtaggtatctcagttcggtgtaggtcgttcgctccaagctgggctgtgtgcacgaaccccccgttcagcccgaccgctgcgccttatccggtaactatcgtcttgagtccaacccggtaagacacgacttatcgccactggcagcagccactggtaacaggattagcagagcgaggtatgtaggcggtgctacagagttcttgaagtggtggcctaactacggctacactagaagaacagtatttggtatctgcgctctgctgaagccagttaccttcggaaaaagagttggtagctcttgatccggcaaacaaaccaccgctggtagcggtggtttttttgtttgcaagcagcagattacgcgcagaaaaaaaggatctcaagaagatcctttgatcttttctacggggtctgacgctcagtggaacgaaaactcacgttaagggattttggtcatgagattatcaaaaaggatcttcacctagatccttttaaattaaaaatgaagttttaaatcaatctaaagtatatatgagtaaacttggtctgacagttaccaatgcttaatcagtgaggcacctatctcagcgatctgtctatttcgttcatccatagttgcctgactccccgtcgtgtagataactacgatacgggagggcttaccatctggccccagtgctgcaatgataccgcgagacccacgctcaccggctccagatttatcagcaataaaccagccagccggaagggccgagcgcagaagtggtcctgcaactttatccgcctccatccagtctattaattgttgccgggaagctagagtaagtagttcgccagttaatagtttgcgcaacgttgttgccattgctacaggcatcgtggtgtcacgctcgtcgtttggtatggcttcattcagctccggttcccaacgatcaaggcgagttacatgatcccccatgttgtgcaaaaaagcggttagctccttcggtcctccgatcgttgtcagaagtaagttggccgcagtgttatcactcatggttatggcagcactgcataattctcttactgtcatgccatccgtaagatgcttttctgtgactggtgagtactcaaccaagtcattctgagaatagtgtatgcggcgaccgagttgctcttgcccggcgtcaatacgggataataccgcgccacatagcagaactttaaaagtgctcatcattggaaaacgttcttcggggcgaaaactctcaaggatcttaccgctgttgagatccagttcgatgtaacccactcgtgcacccaactgatcttcagcatcttttactttcaccagcgtttctgggtgagcaaaaacaggaaggcaaaatgccgcaaaaaagggaataagggcgacacggaaatgttgaatactcatactcttcctttttcaatattattgaagcatttatcagggttattgtctcatgagcggatacatatttgaatgtatttagaaaaataaacaaataggggttccgcgcacatttccccgaaaagtgccacctgacgtctaagaaaccattattatcatgacattaacctataaaaataggcgtatcacgaggccctttcgtctcgcgcgtttcggtgatgacggtgaaaacctctgacacatgcagctcccggagacggtcacagcttgtctgtaagcggatgccgggagcagacaagcccgtcagggcgcgtcagcgggtgttggcgggtgtcggggctggcttaactatgcggcatcagagcagattgtactgagagtgcaccatatgcggtgtgaaataccgcacagatgcgtaaggagaaaataccgcatcaggcgccattcgccattcaggctgcgcaactgttgggaagggcgatcggtgcgggcctcttcgctattacgccagctggcgaaagggggatgtgctgcaaggcgattaagttgggtaacgccagggttttcccagtcacgacgttgtaaaacgacggccagtgaattcgagctcggtacc

SEQ ID NO: 88 - DNA, 60 bp, Artificial
  Artificial DNA Sequence
tcctctatatacacaactggggatccaccatgtcgaggttccagtctcttttcttcttcg

SEQ ID NO: 89 - DNA, 53 bp, Artificial
  Artificial DNA Sequence
tctagatctcgagctcgctagagtcgacctagaggtcgctcgggtcgagcgcg

SEQ ID NO: 90 - DNA, 55 bp, Artificial
  Artificial DNA Sequence
tcctctatatacacaactggggatccaccatgaggtccttcatcagcgccgcgac

SEQ ID NO: 91 - DNA, 53 bp, Artificial
  Artificial DNA Sequence
tctagatctcgagctcgctagagtcgacctacgccttgaccagccactcgccc

SEQ ID NO: 92 - DNA, 1557 bp, Pycnoporus cinnabarinus
atgtcgaggttccagtccctcttcttcttcgtcctcgtctccctcaccgctgtggccaacgcagccatagggcctgtggcggacctgacccttaccaatgcccaggtcagccccgatggcttcgctcgcgaggccgtcgtggtgaacggtatcacccctgcccctctcatcacaggcaataagggcgatcgattccagctcaatgtcatcgaccagttgacaaatcataccatgttgaaaacatctagtattcattggcacggcttcttccagcaaggcacgaactgggccgatggtcccgcgttcgtgaaccagtgtcccatcgcttcgggccactcgttcttgtatgactttcaagttcccgaccaagcagggactttctggtaccatagccatctctccacgcaatactgcgatggtttgagggggcctttcgtcgtctacgaccccaacgatcctcacgctagcctgtatgacattgataacgacgacactgtcattacgctggctgattggtatcacgttgctgccaagctcggacctcgcttcccatttggctccgattcaacccttatcaatggacttggtcgaaccactggcatagcaccgtccgacttggcagttatcaaggtcacgcagggcaagcgctaccgcttccgcttggtgtcgctttcttgcgatccgaaccatacattcagcattgataatcacacaatgactataattgaggcggactcgatcaacactcaacccctagaggttgattcaatccagatttttgccgcgcagcgctactccttcgtgctggatgctagccagccggtggataactactggatccgcgcaaaccctgccttcggaaacacaggttttgctggtggaatcaattctgccatcctgcgttatgatggcgcacccgagatcgagcctacgtctgtccagactactcctacgaagcctctgaacgaggtcgacttgcatcctctctcgcctatgcctgtgcctggcagccccgagcccggaggtgtcgacaagcctctgaacttggtcttcaacttcaacggcaccaacttcttcatcaacgaccacacctttgtcccgccgtctgtcccagtcttgctacaaatcctcagtggggcgcaggcggctcaggacctggtcccggagggcagcgtgttcgttcttcccagcaactcgtccattgagatatccttccctgccactgccaatgcccctggattcccccatccgttccacttgcacggtcacgccttcgctgtcgtccggagcgccgggagcagcgtctacaactacgacaacccgatcttccgcgacgtcgtcagcaccggccagcccggcgacaacgtcacgattcgcttcgagaccaataacccaggcccgtggttcctccactgccacattgacttccacctcgacgcaggctttgctgtagtcatggccgaggacactccggacaccaaggccgcgaaccctgttcctcaggcgtggtcggacttgtgccccatctatgatgcacttgaccccagcgacctctag

SEQ ID NO: 93 - protein, 518 aa, Pycnoporus cinnabarinus; identical to SEQ ID NO: 52

SEQ ID NO: 94 - DNA, 1863 bp, Myceliophthora thermophila
atgaggtccttcatcagcgccgcgacgcttttggtgggcattctcacccctagcgttgctgctgcccctccatccacccctgagcagcgcgacctgctcgtcccgatcacggagagggaggaggcagccgtgaaggctcgccagcagagctgcaacacccccagcaaccgggcgtgctggactgacggatacgacatcaacaccgactacgaagtggacagcccggacacgggtgttgttcggccttatactctgactctcaccgaagtcgacaactggaccggacctgatggcgtcgtcaaggagaaggtcatgctggttaacaatagtataatcggaccaacaatctttgcggactggggcgacacgatccaggtaacggtcatcaacaacctcgagaccaacggcacgtcgatccactggcacggactgcaccagaagggcaccaacctgcacgacggcgccaacggtatcaccgagtgcccgatcccgcccaagggagggaggaaggtgtaccggttcaaggctcagcagtacgggacgagctggtaccactcgcacttctcggcccagtacggcaacggcgtggtcggggccattcagatcaacgggccggcctcgctgccgtacgacaccgacctgggcgtgttccccatcagcgactactactacagctcggccgacgagctggtggaactcaccaagaactcgggcgcgcccttcagcgacaacgtcctgttcaacggcacggccaagcacccggagacgggcgagggcgagtacgccaacgtgacgctcaccccgggccggcggcaccgcctgcgcctgatcaacacgtcggtcgagaaccacttccaggtctcgctcgtcaaccacaccatgaccatcatcgccgccgacatggtgcccgtcaacgccatgacggtcgacagcctcttcctcggcgtcggccagcgctacgatgtcgtcatcgaagccagccgaacgcccgggaactactggtttaacgtcacatttggcggcggcctgctctgcggcggctccaggaatccctacccggccgccatcttccactacgccggcgcccccggcggcccgcccacggacgagggcaaggccccggtcgaccacaactgcctggacctccccaacctcaagcccgtcgtggcccgcgacgtgcccctgagcggcttcgccaagcggcccgacaacacgctcgacgtcaccctcgacaccacgggcacgcccctgttcgtctggaaggtcaacggcagcgccatcaacatcgactggggcaggcccgtcgtcgactacgtcctcacgcagaacaccagcttcccacccgggtacaacattgtcgaggtgaacggagctgatcagtggtcgtactggttgatcgagaacgatcccggcgcacctttcaccctaccgcatccgatgcacctgcacggccacgacttttacgtgctgggccgctcgcccgacgagtcgccggcatccaacgagcggcacgtgttcgatccggcgcgggacgcgggcctgctgagcggggccaaccctgtgcggcgggacgtgacgatgctgccggcgttcgggtgggtggtgctggccttccgggccgacaacccgggcgcctggctgttccactgccacatcgcctggcacgtctcgggcggcctgggcgtcgtctacctcgagcgcgccgacgacctgcgcggggccgtctcggacgccgacgccgacgacctcgaccgcctctgcgccgactggcgccgctactggcctaccaacccctaccccaagtccgactcgggcctcaagcaccgctgggtcgaggagggcgagtggctggtcaaggcgtag

SEQ ID NO: 95 - protein, 620 aa, Myceliophthora thermophila
MRSFISAATLLVGILTPSVAAAPPSTPEQRDLLVPITEREEAAVKARQQSCNTPSNRACWTDGYDINTDYEVDSPDTGVVRPYTLTLTEVDNWTGPDGVVKEKVMLVNNSIIGPTIFADWGDTIQVTVINNLETNGTSIHWHGLHQKGTNLHDGANGITECPIPPKGGRKVYRFKAQQYGTSWYHSHFSAQYGNGVVGAIQINGPASLPYDTDLGVFPISDYYYSSADELVELTKNSGAPFSDNVLFNGTAKHPETGEGEYANVTLTPGRRHRLRLINTSVENHFQVSLVNHTMTIIAADMVPVNAMTVDSLFLGVGQRYDVVIEASRTPGNYWFNVTFGGGLLCGGSRNPYPAAIFHYAGAPGGPPTDEGKAPVDHNCLDLPNLKPVVARDVPLSGFAKRPDNTLDVTLDTTGTPLFVWKVNGSAINIDWGRPVVDYVLTQNTSFPPGYNIVEVNGADQWSYWLIENDPGAPFTLPHPMHLHGHDFYVLGRSPDESPASNERHVFDPARDAGLLSGANPVRRDVTMLPAFGWVVLAFRADNPGAWLFHCHIAWHVSGGLGVVYLERADDLRGAVSDADADDLDRLCADWRRYWPTNPYPKSDSGLKHRWVEEGEWLVKA